European Patent Application EP 4 560 015 A2, published May 28, 2025. Title: Modified polyketide synthase enzymes and uses thereof. Applicant: BGENE GENETICS. The sequence listing filed with the application follows.

SEQUENCE LISTING (46 sequences)

SEQ ID NO: 1 - protein, 394 aa, Piper methysticum
MSKTVEEIWAAQRARGPATVLAIGTAAPANVVYQADYPDYYFRITKSEHMTELKEKFRRMCDKSMITKRHMHLSEELLKNNPDICAYMAPSLDARQDMVVVEVPKLGKEAAAKAIKEWGRPKSAITHLIFCTTSGVDMPGADFQLTKLLGLCPSVRRTMLYQQGCFAGGTVLRLAKDLAENNAGARVLVVCSEITAVTFRGPSETHLDSMVGQALFGDGASAIIVGADPDPVIERPLFQIVSAAQTILPDSDGAIDGHLREVGLTFHLLKDVPGLISKNIEKSLKEAFAPLGIDDWNSIFWIVHPGGPAILDQVEAKLRLKVEKLKTTRTVLSEYGNMSSACVLFILDEMRRNSMEEGKATTGEGLHWGVLFGFGPGLTVETVVLHSLPIAEAN

SEQ ID NO: 2 - protein, 394 aa, Elaeis guineensis
MAKVLLEEIRSSQRAEGPATILAIGTATPANVVYQADYPDYYFRITKSEHLTDLKEKFKRMCDKSMIRKRYMHLSEEILKENPNICAYMAPSLDARQDVVVVEVPKLGKEAAVKAIKEWGQPKSKITHLVFCTTSGVDMPGADYQLTKLLGLRPSVNRLMMYQQGCFAGGTVLRLAKDLAENNRGARVLVVCSEITAVTFRGPSESHLDSLVGQALFGDGAAAIIVGADPDPAIERPLFQLVSASQTILPDSEGAIDGHLREVGLTFHLLKDVPGLISKNIHKSLVEAFVPLGISDWNSIFWIAHPGGPAILDQVEAKLGLEKEKMRATRHVLSEYGNMSSACVLFILDEMRRRSAEEGKATTGEGLEWGVLFGFGPGLTVETVVLHSLPISTR

SEQ ID NO: 3 - protein, 393 aa, Vitis vinifera
MVSVGEIRKSQRAEGPATVLAIGTATPANCVYQADYPDYYFRITNSEHMTELKEKFKRMCDKSMINKRYMHLNEEILKENPNVCAYMAPSLDARQDMVVVEVPKLGKEAAVKAIKEWGQPKSKITHLVFCTTSGVDMPGADYQLTKLLGLKPSVKRLMMYQQGCFAGGTVLRLAKDLAENNAGARVLVVCSEITAVTFRGPSDTHLDSLVGQALFGDGAAAIIIGADPDTKIERPLFELVSAAQTILPDSEGAIDGHLREVGLTFHLLKDVPGLISKNIEKSLVEAFKPIGISDWNSLFWIAHPGGPAILDQVELKLGLKEEKLRATRHVLSEYGNMSSACVLFILDEMRKKSIEEGKGTTGEGLEWGVLFGFGPGLTVETVVLHSLATQSTH

SEQ ID NO: 4 - protein, 394 aa, synthetic construct
MSKTVEEIWAAQRARGPATVLAIGTAAPANVVYQADYADYYFRITKSEHMTELKEKFRRMCDKSMITKRHMHLSEELLKNNPDICAYMAPSLDARQDMVVVEVPKLGKEAAAKAIKEWGRPKSAITHLIFCTTSGVDMPGADFQLTKLLGLCPSVRRTMLYQQGCFAGGTVLRLAKDLAENNAGARVLVVCSEITAVTFRGPSETHLDSMVGQALFGDGASAIIVGADPDPVIERPLFQIVSAAQTILPDSDGAIDGHLREVGLTFHLLKDVPGLISKNIEKSLKEAFAPLGIDDWNSIFWIVHPGGPAILDQVEAKLRLKVEKLKTTRTVLSEYGNMSSACVLFILDEMRRNSMEEGKATTGEGLHWGVLFGFGPGLTVETVVLHSLPIAEAN

SEQ ID NO: 5 - protein, 394 aa, Rheum palmatum
MSKTVEEIWAAQRARGPATVLAIGTAAPANVVYQADYPDYYFRITKSEHMTELKEKFRRMCDKSMITKRHMHLSEELLKNNPDICAYMAPSLDARQDMVVVEVPKLGKEAAAKAIKEWGRPKSAITHLIFCTTSGVDMPGADFQLTKLLGLCPSVRRTMLYQQGCFAGGTVLRLAKDLAENNAGARVLVVCSEITAVTFRGPSETHLDSMVGQALFGDGASAIIVGADPDPVIERPLFQIVSAAQTILPDSDGAIDGHLREVGLTFHLLKDVPGLISKNIEKSLKEAFAPLGIDDWNSIFWIVHPGGPAILDQVEAKLRLKPEKLKTTRTVLSEYGNMSSACVLFILDEMRRNSMEEGKATTGEGLHWGVLFGFGPGLTVETVVLHSLPIAEAN

SEQ ID NO: 6 - protein, 394 aa, synthetic construct
MAKVLLEEIRSSQRAEGPATILAIGTATPANVVYQADYADYYFRITKSEHLTDLKEKFKRMCDKSMIRKRYMHLSEEILKENPNICAYMAPSLDARQDVVVVEVPKLGKEAAVKAIKEWGQPKSKITHLVFCTTSGVDMPGADYQLTKLLGLRPSVNRLMMYQQGCFAGGTVLRLAKDLAENNRGARVLVVCSEITAVTFRGPSESHLDSLVGQALFGDGAAAIIVGADPDPAIERPLFQLVSASQTILPDSEGAIDGHLREVGLTFHLLKDVPGLISKNIHKSLVEAFVPLGISDWNSIFWIAHPGGPAILDQVEAKLGLEKEKMRATRHVLSEYGNMSSACVLFILDEMRRRSAEEGKATTGEGLEWGVLFGFGPGLTVETVVLHSLPISTR

SEQ ID NO: 7 - protein, 393 aa, synthetic construct
MVSVGEIRKSQRAEGPATVLAIGTATPANCVYQADYADYYFRITNSEHMTELKEKFKRMCDKSMINKRYMHLNEEILKENPNVCAYMAPSLDARQDMVVVEVPKLGKEAAVKAIKEWGQPKSKITHLVFCTTSGVDMPGADYQLTKLLGLKPSVKRLMMYQQGCFAGGTVLRLAKDLAENNAGARVLVVCSEITAVTFRGPSDTHLDSLVGQALFGDGAAAIIIGADPDTKIERPLFELVSAAQTILPDSEGAIDGHLREVGLTFHLLKDVPGLISKNIEKSLVEAFKPIGISDWNSLFWIAHPGGPAILDQVELKLGLKEEKLRATRHVLSEYGNMSSACVLFILDEMRKKSIEEGKGTTGEGLEWGVLFGFGPGLTVETVVLHSLATQSTH

SEQ ID NO: 8 - protein, 393 aa, synthetic construct
MVSVGEIRKSQRAEGPATVLAIGTATPANCVYQADYPDYYFRITNSEHMTELKEKFKRMCDKSQINKRYMHLNEEILKENPNVCAYMAPSLDARQDMVVVEVPKLGKEAAVKAIKEWGQPKSKITHLVFCTTSGVDMPGADYQLTKLLGLKPSVKRLMMYQQGCFAGGTVLRLAKDLAENNAGARVLVVCSEITAVTFRGPSDTHLDSLVGQALFGDGAAAIIIGADPDTKIERPLFELVSAAQTILPDSEGAIDGHLREVGLTFHLLKDVPGLISKNIEKSLVEAFKPIGISDWNSLFWIAHPGGPAILDQVELKLGLKEEKLRATRHVLSEYGNMSSACVLFILDEMRKKSIEEGKGTTGEGLEWGVLFGFGPGLTVETVVLHSLATQSTH

SEQ ID NO: 9 - protein, 384 aa, Rheum palmatum
MATEEMKKLATVMAIGTANPPNCYYQADFPDFYFRVTNSDHLINLKQKFKRLCENSRIEKRYLHVTEEILKENPNIAAYEATSLNVRHKMQVKGVAELGKEAALKAIKEWGQPKSKITHLIVCCLAGVDMPGADYQLTKLLDLDPSVKRFMFYHLGCYAGGTVLRLAKDIAENNKGARVLIVCSEMTTTCFRGPSETHLDSMIGQAILGDGAAAVIVGADPDLTVERPIFELVSTAQTIVPESHGAIEGHLLESGLSFHLYKTVPTLISNNIKTCLSDAFTPLNISDWNSLFWIAHPGGPAILDQVTAKVGLEKEKLKVTRQVLKDYGNMSSATVFFIMDEMRKKSLENGQATTGEGLEWGVLFGFGPGITVETVVLRSVPVIS

SEQ ID NO: 10 - protein, 394 aa, synthetic construct
MSKTVEEIWAAQRARGPATVLAIGTAAPANVVYQADYADYYFRITKSEHMTELKEKFRRMCDKSMITKRHMHLSEELLKNNPDICAYMAPSLDARQDMVVVEVPKLGKEAAAKAIKEWGRPKSAITHLIFCTTSGVDMPGADFQLTKLLGLCPSVRRTMLYQQGCFAGGTVLRLAKDLAENNAGARVLVVCSEITAVTFRGPSETHLDSMVGQALFGDGASAIIVGADPDPVIERPLFQIVSAAQTILPDSDGAIDGHLREVGLTFHLLKDVPGLISKNIEKSLKEAFAPLGIDDWNSIFWIVHPGGPAILDQVEAKLRLKPEKLKTTRTVLSEYGNMSSACVLFILDEMRRNSMEEGKATTGEGLHWGVLFGFGPGLTVETVVLHSLPIAEAN

SEQ ID NO: 11 - protein, 393 aa, synthetic construct
MVSVGEIRKSQRAEGPATVLAIGTATPANCVYQADYADYYFRITNSEHMTELKEKFKRMCDKSQINKRYMHLNEEILKENPNVCAYMAPSLDARQDMVVVEVPKLGKEAAVKAIKEWGQPKSKITHLVFCTTSGVDMPGADYQLTKLLGLKPSVKRLMMYQQGCFAGGTVLRLAKDLAENNAGARVLVVCSEITAVTFRGPSDTHLDSLVGQALFGDGAAAIIIGADPDTKIERPLFELVSAAQTILPDSEGAIDGHLREVGLTFHLLKDVPGLISKNIEKSLVEAFKPIGISDWNSLFWIAHPGGPAILDQVELKLGLKEEKLRATRHVLSEYGNMSSACVLFILDEMRKKSIEEGKGTTGEGLEWGVLFGFGPGLTVETVVLHSLATQSTH

SEQ ID NO: 12 - protein, 394 aa, synthetic construct
MSKTVEEIWAAQRARGPATVLAIGTAAPANVVYQADYPDYYFRITKSEHMTELKEKFRRMCDKSQITKRHMHLSEELLKNNPDICAYMAPSLDARQDMVVVEVPKLGKEAAAKAIKEWGRPKSAITHLIFCTTSGVDMPGADFQLTKLLGLCPSVRRTMLYQQGCFAGGTVLRLAKDLAENNAGARVLVVCSEITAVTFRGPSETHLDSMVGQALFGDGASAIIVGADPDPVIERPLFQIVSAAQTILPDSDGAIDGHLREVGLTFHLLKDVPGLISKNIEKSLKEAFAPLGIDDWNSIFWIVHPGGPAILDQVEAKLRLKVEKLKTTRTVLSEYGNMSSACVLFILDEMRRNSMEEGKATTGEGLHWGVLFGFGPGLTVETVVLHSLPIAEAN

SEQ ID NO: 13 - protein, 394 aa, synthetic construct
MAKVLLEEIRSSQRAEGPATILAIGTATPANVVYQADYPDYYFRITKSEHLTDLKEKFKRMCDKSMIRKRYMHLSEEILKENPNICAYMAPSLDARQDVVVVEVPKLGKEAAVKAIKEWGQPKSKITHLVFCTTSGVDMPGADYQLTKLLGLRPSVNRLMMYQQGCFAGGTVLRLAKDLAENNRGARVLVVCSEITAVTFRGPSESHLDSLVGQALFGDGAAAIIVGADPDPAIERPLFQLVSASQTILPDSEGAIDGHLREVGLTFHLLKDVPGLISKNIHKSLVEAFAPLGISDWNSIFWIAHPGGPAILDQVEAKLGLEKEKMRATRHVLSEYGNMSSACVLFILDEMRRRSAEEGKATTGEGLEWGVLFGFGPGLTVETVVLHSLPISTR

SEQ ID NO: 14 - protein, 394 aa, synthetic construct
MAKVLLEEIRSSQRADGPATILAIGTATPANVVYQADYPDYYFRITKSEHLTDLKEKFKRMCDKSMIRKRYMHLSEEILKENPNICAYMAPSLDARQDVVVVEVPKLGKEAAVKAIKEWGQPKSKITHLVFCTTSGVDMPGADYQLTKLLGLRPSVNRLMMYQQGCFAGGTVLRLAKDLAENNRGARVLVVCSEITAVTFRGPSESHLDSLVGQALFGDGAAAIIVGADPDPAIERPLFQLVSASQTILPDSEGAIDGHLREVGLTFHLLKDVPGLISKNIHKSLVEAFVPLGISDWNSIFWIAHPGGPAILDQVEAKLGLEKEKMRATRHVLSEYGNMSSACVLFILDEMRRRSAEEGKATTGEGLEWGVLFGFGPGLTVETVVLHSLPISTR

SEQ ID NO: 15 - protein, 393 aa, synthetic construct
MVSVGEIRKSQRAEGPATVLAIGTATPANCVYQADYPDYYFRITNSEHMTELKEKFKRMCDKSMINKRYMHLNEEILKENPNVCAYMAPSLDARQDMVVVEVPKLGKEAAVKAIKEWGQPKSKITHLVFCTTSGVDMPGADYQLTKLLGLKPSVKRLMMYQQGCFAGGTVLRLAKDLAENNAGARVLVVCSEITAVTFRGPSDTHLDSLVGQALFGDGAAAIIIGADPDTKIERPLFELVSAAQTILPDSEGAIDGHLREVGLTFHLLKDVPGLISKNIEKSLVEAFAPIGISDWNSLFWIAHPGGPAILDQVELKLGLKEEKLRATRHVLSEYGNMSSACVLFILDEMRKKSIEEGKGTTGEGLEWGVLFGFGPGLTVETVVLHSLATQSTH

SEQ ID NO: 16 - DNA, 1185 bp, Piper methysticum
  source 1..1185: mol_type = other DNA
atgtccaaaaccgttgaagagatctgggcagcccaacgcgctcgaggcccagctacagtgcttgcgatcggcaccgctgctcccgccaacgtggtgtaccaggcggactacccagactattatttccgcattaccaagagcgagcatatgaccgaattgaaggaaaagtttcgccggatgtgcgataagagtatgatcaccaagcgccatatgcatctgagtgaagagcttctgaaaaacaaccccgacatctgcgcgtacatggcgccctcgctcgacgcgcgtcaggacatggtggtggtggaagttccaaagctggggaaggaggctgccgcaaaagccatcaaagagtggggccggccgaagagcgccatcacccacctgattttctgcaccaccagcggcgtggacatgccgggcgccgacttccaactgactaagctgctcggcctatgcccgtcggtgcgccgcaccatgctgtaccagcaggggtgcttcgcgggcggtacagtgctgcgcctggccaaggatctggcggaaaacaatgcgggcgcccgcgtcctggtggtctgctcggaaatcaccgccgtgactttccgcggcccgtccgaaacccacctcgattcaatggttggccaggccttgtttggtgacggcgcctccgcgattatcgtgggcgccgacccggacccggtgattgagcgccctctcttccagatcgtctcggccgcccagaccattctgccggattcggacggtgcgatcgacgggcacctgcgggaggtgggcctgacctttcacctgctgaaggacgtaccgggcctgatcagcaagaacatcgagaagagcttgaaagaggccttcgccccgttaggcatcgacgattggaactcgatcttctggatcgtgcacccgggtggccctgcaatcctggatcaggtagaagccaagctccgtctgaaggtcgaaaagttgaaaaccaccaggacggtcctgtctgagtacgggaacatgagcagcgcctgtgtcttgttcatcctggatgagatgcgtcgtaacagcatggaagagggtaaagccacgactggcgaaggtctgcactggggcgtcctgttcgggttcggccccggactgacggtagagacggtcgtcctgcacagcttgcccatagcagaggcaaattga

SEQ ID NO: 17 - DNA, 1185 bp, Elaeis guineensis
  source 1..1185: mol_type = other DNA
atggccaaggtcttgttggaggaaatccgctcctcgcagcgcgccgaaggccccgccaccatcttggccatcggcacggctaccccggcgaacgtggtgtatcaggcagactacccagactactacttccgtattaccaagagcgagcatttgaccgaccttaaagaaaaatttaagcgtatgtgcgacaagtccatgattcgcaagcgctacatgcacctgagtgaagagatcttgaaggagaatccaaacatttgtgcctacatggcccccagtctcgacgctcgccaggacgtcgtagtcgtcgaggtgccgaagctgggcaaggaggcggcggtgaaggccatcaaggaatggggccaaccgaagtcgaagatcacccacctggtattttgcacgacgtccggcgtggacatgccgggtgcggactatcagctgactaagcttctgggcctgaggccaagcgtcaacaggctgatgatgtaccagcagggctgcttcgccggcggcacagtgctacgtctcgccaaagacttggccgaaaacaatcgtggtgcgcgcgtgctggtcgtgtgtagcgagatcaccgctgtgacgtttcgcggtccatccgagagccatctggacagcctggtcggccaggcgctgttcggtgatggcgccgccgcgatcatcgtgggcgcggacccggacccggccattgagcgccccctgttccagttggtgtcggccagccagaccatccttccagactcggagggcgcgattgacggccacctgcgggaagtgggactcaccttccacttactcaaagacgtaccaggcctgatctctaagaacatccataagtccctggtggaggccttcgtgccgctgggcatcagcgattggaacagtattttctggatcgcccaccctggtggtccggctatcctggaccaggtggaagccaagcttggcttggaaaaagagaagatgcgagccacccgccacgtgctgagcgaatacggcaacatgtccagcgcctgcgtgctgttcatcctcgacgagatgcgacgtcgcagcgcagaagaggggaaagccaccacaggtgagggcctcgagtggggtgtgttgttcggtttcgggccgggccttaccgtggagaccgtggtgctgcacagtcttccgataagtacccgttga

SEQ ID NO: 18 - DNA, 1182 bp, Vitis vinifera
  source 1..1182: mol_type = other DNA
atggtttctgtgggcgaaatccgcaagagccagcgtgcagagggcccggcaactgtactcgccatcggcaccgccacgcccgccaactgcgtgtaccaggcggactacccggactactacttccgaatcaccaacagtgaacacatgactgagctaaaagagaagttcaaacgtatgtgcgataagagcatgatcaacaagcgctacatgcacctgaacgaggagatccttaaggagaaccccaacgtttgcgcgtacatggccccgtcgctggacgctcgccaggatatggtggtggtggaggtgccaaaattgggcaaggaagcggccgtaaaggctattaaggagtggggtcagcctaagagcaagatcacgcatctggttttctgcacgaccagcggcgtggatatgcctggtgccgactatcagttgacgaagcttctgggtttgaagccgagcgtaaaacgcctcatgatgtatcagcagggctgtttcgccggcgggaccgtgttgcgcttggctaaagacctcgctgagaataacgccggcgcccgcgtgctcgtggtctgctcagagattaccgccgtcaccttccgtgggccctcggatacccacctggatagcttggtgggtcaggccctgttcggtgacggcgccgcggccattattatcggcgcggacccggacacaaagatcgaacgccccctgttcgaactggtctccgcggcccaaaccatccttccggatagcgaaggtgccatcgacggccacctgcgggaagtcggtctgaccttccacctgctgaaagacgtcccgggcctgatctcgaaaaacatcgagaaatcgctggtcgaggcgttcaagccgatcggcatctccgactggaattcgctgttctggatcgcgcatccaggcggcccggccatcctggaccaagtggagctcaagctgggcctgaaggaggagaagctgcgggccaccaggcatgtgctgtccgaatatgggaacatgagctccgcatgcgtcctgtttattctggacgaaatgcgcaagaagtcgatagaagaaggcaaggggaccacaggcgaagggctggaatggggcgtgctgtttggctttggcccaggactgaccgtcgaaaccgtcgtgctgcacagcctggcaacccaaagtacccactga

SEQ ID NO: 19 - DNA, 1185 bp, synthetic construct
  source 1..1185: mol_type = other DNA
atgtccaaaaccgttgaagagatctgggcagcccaacgcgctcgaggcccagctacagtgcttgcgatcggcaccgctgctcccgccaacgtggtgtaccaggcggactacgcagactattatttccgcattaccaagagcgagcatatgaccgaattgaaggaaaagtttcgccggatgtgcgataagagtatgatcaccaagcgccatatgcatctgagtgaagagcttctgaaaaacaaccccgacatctgcgcgtacatggcgccctcgctcgacgcgcgtcaggacatggtggtggtggaagttccaaagctggggaaggaggctgccgcaaaagccatcaaagagtggggccggccgaagagcgccatcacccacctgattttctgcaccaccagcggcgtggacatgccgggcgccgacttccaactgactaagctgctcggcctatgcccgtcggtgcgccgcaccatgctgtaccagcaggggtgcttcgcgggcggtacagtgctgcgcctggccaaggatctggcggaaaacaatgcgggcgcccgcgtcctggtggtctgctcggaaatcaccgccgtgactttccgcggcccgtccgaaacccacctcgattcaatggttggccaggccttgtttggtgacggcgcctccgcgattatcgtgggcgccgacccggacccggtgattgagcgccctctcttccagatcgtctcggccgcccagaccattctgccggattcggacggtgcgatcgacgggcacctgcgggaggtgggcctgacctttcacctgctgaaggacgtaccgggcctgatcagcaagaacatcgagaagagcttgaaagaggccttcgccccgttaggcatcgacgattggaactcgatcttctggatcgtgcacccgggtggccctgcaatcctggatcaggtagaagccaagctccgtctgaaggtcgaaaagttgaaaaccaccaggacggtcctgtctgagtacgggaacatgagcagcgcctgtgtcttgttcatcctggatgagatgcgtcgtaacagcatggaagagggtaaagccacgactggcgaaggtctgcactggggcgtcctgttcgggttcggccccggactgacggtagagacggtcgtcctgcacagcttgcccatagcagaggcaaattga

SEQ ID NO: 20 - DNA, 1185 bp, synthetic construct
  source 1..1185: mol_type = other DNA
atgtccaaaaccgttgaagagatctgggcagcccaacgcgctcgaggcccagctacagtgcttgcgatcggcaccgctgctcccgccaacgtggtgtaccaggcggactacccagactattatttccgcattaccaagagcgagcatatgaccgaattgaaggaaaagtttcgccggatgtgcgataagagtatgatcaccaagcgccatatgcatctgagtgaagagcttctgaaaaacaaccccgacatctgcgcgtacatggcgccctcgctcgacgcgcgtcaggacatggtggtggtggaagttccaaagctggggaaggaggctgccgcaaaagccatcaaagagtggggccggccgaagagcgccatcacccacctgattttctgcaccaccagcggcgtggacatgccgggcgccgacttccaactgactaagctgctcggcctatgcccgtcggtgcgccgcaccatgctgtaccagcaggggtgcttcgcgggcggtacagtgctgcgcctggccaaggatctggcggaaaacaatgcgggcgcccgcgtcctggtggtctgctcggaaatcaccgccgtgactttccgcggcccgtccgaaacccacctcgattcaatggttggccaggccttgtttggtgacggcgcctccgcgattatcgtgggcgccgacccggacccggtgattgagcgccctctcttccagatcgtctcggccgcccagaccattctgccggattcggacggtgcgatcgacgggcacctgcgggaggtgggcctgacctttcacctgctgaaggacgtaccgggcctgatcagcaagaacatcgagaagagcttgaaagaggccttcgccccgttaggcatcgacgattggaactcgatcttctggatcgtgcacccgggtggccctgcaatcctggatcaggtagaagccaagctccgtctgaagccggaaaagttgaaaaccaccaggacggtcctgtctgagtacgggaacatgagcagcgcctgtgtcttgttcatcctggatgagatgcgtcgtaacagcatggaagagggtaaagccacgactggcgaaggtctgcactggggcgtcctgttcgggttcggccccggactgacggtagagacggtcgtcctgcacagcttgcccatagcagaggcaaattga

SEQ ID NO: 21 - DNA, 1185 bp, synthetic construct
  source 1..1185: mol_type = other DNA
atggccaaggtcttgttggaggaaatccgctcctcgcagcgcgccgaaggccccgccaccatcttggccatcggcacggctaccccggcgaacgtggtgtatcaggcagactacgcagactactacttccgtattaccaagagcgagcatttgaccgaccttaaagaaaaatttaagcgtatgtgcgacaagtccatgattcgcaagcgctacatgcacctgagtgaagagatcttgaaggagaatccaaacatttgtgcctacatggcccccagtctcgacgctcgccaggacgtcgtagtcgtcgaggtgccgaagctgggcaaggaggcggcggtgaaggccatcaaggaatggggccaaccgaagtcgaagatcacccacctggtattttgcacgacgtccggcgtggacatgccgggtgcggactatcagctgactaagcttctgggcctgaggccaagcgtcaacaggctgatgatgtaccagcagggctgcttcgccggcggcacagtgctacgtctcgccaaagacttggccgaaaacaatcgtggtgcgcgcgtgctggtcgtgtgtagcgagatcaccgctgtgacgtttcgcggtccatccgagagccatctggacagcctggtcggccaggcgctgttcggtgatggcgccgccgcgatcatcgtgggcgcggacccggacccggccattgagcgccccctgttccagttggtgtcggccagccagaccatccttccagactcggagggcgcgattgacggccacctgcgggaagtgggactcaccttccacttactcaaagacgtaccaggcctgatctctaagaacatccataagtccctggtggaggccttcgtgccgctgggcatcagcgattggaacagtattttctggatcgcccaccctggtggtccggctatcctggaccaggtggaagccaagcttggcttggaaaaagagaagatgcgagccacccgccacgtgctgagcgaatacggcaacatgtccagcgcctgcgtgctgttcatcctcgacgagatgcgacgtcgcagcgcagaagaggggaaagccaccacaggtgagggcctcgagtggggtgtgttgttcggtttcgggccgggccttaccgtggagaccgtggtgctgcacagtcttccgataagtacccgttga

SEQ ID NO: 22 - DNA, 1182 bp, synthetic construct
  source 1..1182: mol_type = other DNA
atggtttctgtgggcgaaatccgcaagagccagcgtgcagagggcccggcaactgtactcgccatcggcaccgccacgcccgccaactgcgtgtaccaggcggactacccggactactacttccgaatcaccaacagtgaacacatgactgagctaaaagagaagttcaaacgtatgtgcgataagagcatgatcaacaagcgctacatgcacctgaacgaggagatccttaaggagaaccccaacgtttgcgcgtacatggccccgtcgctggacgctcgccaggatatggtggtggtggaggtgccaaaattgggcaaggaagcggccgtaaaggctattaaggagtggggtcagcctaagagcaagatcacgcatctggttttctgcacgaccagcggcgtggatatgcctggtgccgactatcagttgacgaagcttctgggtttgaagccgagcgtaaaacgcctcatgatgtatcagcagggctgtttcgccggcgggaccgtgttgcgcttggctaaagacctcgctgagaataacgccggcgcccgcgtgctcgtggtctgctcagagattaccgccgtcaccttccgtgggccctcggatacccacctggatagcttggtgggtcaggccctgttcggtgacggcgccgcggccattattatcggcgcggacccggacacaaagatcgaacgccccctgttcgaactggtctccgcggcccaaaccatccttccggatagcgaaggtgccatcgacggccacctgcgggaagtcggtctgaccttccacctgctgaaagacgtcccgggcctgatctcgaaaaacatcgagaaatcgctggtcgaggcgttcgccccgatcggcatctccgactggaattcgctgttctggatcgcgcatccaggcggcccggccatcctggaccaagtggagctcaagctgggcctgaaggaggagaagctgcgggccaccaggcatgtgctgtccgaatatgggaacatgagctccgcatgcgtcctgtttattctggacgaaatgcgcaagaagtcgatagaagaaggcaaggggaccacaggcgaagggctggaatggggcgtgctgtttggctttggcccaggactgaccgtcgaaaccgtcgtgctgcacagcctggcaacccaaagtacccactga

SEQ ID NO: 23 - DNA, 1182 bp, synthetic construct
  source 1..1182: mol_type = other DNA
atggtttctgtgggcgaaatccgcaagagccagcgtgcagagggcccggcaactgtactcgccatcggcaccgccacgcccgccaactgcgtgtaccaggcggactacccggactactacttccgaatcaccaacagtgaacacatgactgagctaaaagagaagttcaaacgtatgtgcgataagagccagatcaacaagcgctacatgcacctgaacgaggagatccttaaggagaaccccaacgtttgcgcgtacatggccccgtcgctggacgctcgccaggatatggtggtggtggaggtgccaaaattgggcaaggaagcggccgtaaaggctattaaggagtggggtcagcctaagagcaagatcacgcatctggttttctgcacgaccagcggcgtggatatgcctggtgccgactatcagttgacgaagcttctgggtttgaagccgagcgtaaaacgcctcatgatgtatcagcagggctgtttcgccggcgggaccgtgttgcgcttggctaaagacctcgctgagaataacgccggcgcccgcgtgctcgtggtctgctcagagattaccgccgtcaccttccgtgggccctcggatacccacctggatagcttggtgggtcaggccctgttcggtgacggcgccgcggccattattatcggcgcggacccggacacaaagatcgaacgccccctgttcgaactggtctccgcggcccaaaccatccttccggatagcgaaggtgccatcgacggccacctgcgggaagtcggtctgaccttccacctgctgaaagacgtcccgggcctgatctcgaaaaacatcgagaaatcgctggtcgaggcgttcaagccgatcggcatctccgactggaattcgctgttctggatcgcgcatccaggcggcccggccatcctggaccaagtggagctcaagctgggcctgaaggaggagaagctgcgggccaccaggcatgtgctgtccgaatatgggaacatgagctccgcatgcgtcctgtttattctggacgaaatgcgcaagaagtcgatagaagaaggcaaggggaccacaggcgaagggctggaatggggcgtgctgtttggctttggcccaggactgaccgtcgaaaccgtcgtgctgcacagcctggcaacccaaagtacccactga

SEQ ID NO: 24 - DNA, 1155 bp, synthetic construct
  source 1..1155: mol_type = other DNA
atggcaactgaggagatgaagaaattggccaccgtgatggccattggcacggccaaccctccgaactgctactaccaggccgactttcccgacttctacttccgcgtcaccaacagcgaccacctcatcaacctcaagcaaaagttcaagcgcctttgtgaaaactcaaggattgagaagcgttaccttcatgtgaccgaagagattctcaaggaaaacccaaacattgctgcctacgaggcaacctcgttgaatgtaagacacaaaatgcaagtgaaaggagttgcagagcttgggaaagaggctgccctcaaggccatcaaagaatggggccaacccaagtccaagatcacacatctcatcgtgtgttgcctagccggcgttgacatgcccggcgcggattatcaactcactaagcttcttgaccttgacccttccgtcaagcgttttatgttttaccacctaggatgctacgctggtggcactgtccttcgccttgcaaaggacatagcggagaacaacaagggagctcgtgttctcatcgtttgctcagagatgacaacaacttgttttcgtgggccatctgaaacccatctggactccatgataggccaagcaatattaggcgatggggctgcagctgtcatagttggcgcagatccagacctaaccgttgagaggcccatattcgagttggtttccacagcccagactattgtacccgaatcccatggtgcaattgagggccacttgcttgaatctggactcagtttccatttgtacaagaccgttcctacactaatctctaacaacattaaaacttgcctttctgatgctttcactcctctaaacattagcgattggaactctcttttctggatcgcacaccctggtggtcctgccatcctagaccaagttactgctaaggttggtcttgaaaaggagaaactcaaggtaactagacaagtgttgaaggactatggaaacatgtcgagtgctacggtgtttttcatcatggatgagatgaggaagaagtcactcgaaaacggtcaagcaaccactggagaagggctcgagtggggtgttttgtttgggttcgggcctggaatcaccgttgaaactgtagtgctacgcagtgtgcccgtaattagctag

SEQ ID NO: 25 - DNA, 1185 bp, synthetic construct
  source 1..1185: mol_type = other DNA
atgtccaaaaccgttgaagagatctgggcagcccaacgcgctcgaggcccagctacagtgcttgcgatcggcaccgctgctcccgccaacgtggtgtaccaggcggactacgcagactattatttccgcattaccaagagcgagcatatgaccgaattgaaggaaaagtttcgccggatgtgcgataagagtatgatcaccaagcgccatatgcatctgagtgaagagcttctgaaaaacaaccccgacatctgcgcgtacatggcgccctcgctcgacgcgcgtcaggacatggtggtggtggaagttccaaagctggggaaggaggctgccgcaaaagccatcaaagagtggggccggccgaagagcgccatcacccacctgattttctgcaccaccagcggcgtggacatgccgggcgccgacttccaactgactaagctgctcggcctatgcccgtcggtgcgccgcaccatgctgtaccagcaggggtgcttcgcgggcggtacagtgctgcgcctggccaaggatctggcggaaaacaatgcgggcgcccgcgtcctggtggtctgctcggaaatcaccgccgtgactttccgcggcccgtccgaaacccacctcgattcaatggttggccaggccttgtttggtgacggcgcctccgcgattatcgtgggcgccgacccggacccggtgattgagcgccctctcttccagatcgtctcggccgcccagaccattctgccggattcggacggtgcgatcgacgggcacctgcgggaggtgggcctgacctttcacctgctgaaggacgtaccgggcctgatcagcaagaacatcgagaagagcttgaaagaggccttcgccccgttaggcatcgacgattggaactcgatcttctggatcgtgcacccgggtggccctgcaatcctggatcaggtagaagccaagctccgtctgaagccggaaaagttgaaaaccaccaggacggtcctgtctgagtacgggaacatgagcagcgcctgtgtcttgttcatcctggatgagatgcgtcgtaacagcatggaagagggtaaagccacgactggcgaaggtctgcactggggcgtcctgttcgggttcggccccggactgacggtagagacggtcgtcctgcacagcttgcccatagcagaggcaaattga

SEQ ID NO: 26 - DNA, 1182 bp, synthetic construct
  source 1..1182: mol_type = other DNA
atggtttctgtgggcgaaatccgcaagagccagcgtgcagagggcccggcaactgtactcgccatcggcaccgccacgcccgccaactgcgtgtaccaggcggactacgccgactactacttccgaatcaccaacagtgaacacatgactgagctaaaagagaagttcaaacgtatgtgcgataagagccagatcaacaagcgctacatgcacctgaacgaggagatccttaaggagaaccccaacgtttgcgcgtacatggccccgtcgctggacgctcgccaggatatggtggtggtggaggtgccaaaattgggcaaggaagcggccgtaaaggctattaaggagtggggtcagcctaagagcaagatcacgcatctggttttctgcacgaccagcggcgtggatatgcctggtgccgactatcagttgacgaagcttctgggtttgaagccgagcgtaaaacgcctcatgatgtatcagcagggctgtttcgccggcgggaccgtgttgcgcttggctaaagacctcgctgagaataacgccggcgcccgcgtgctcgtggtctgctcagagattaccgccgtcaccttccgtgggccctcggatacccacctggatagcttggtgggtcaggccctgttcggtgacggcgccgcggccattattatcggcgcggacccggacacaaagatcgaacgccccctgttcgaactggtctccgcggcccaaaccatccttccggatagcgaaggtgccatcgacggccacctgcgggaagtcggtctgaccttccacctgctgaaagacgtcccgggcctgatctcgaaaaacatcgagaaatcgctggtcgaggcgttcaagccgatcggcatctccgactggaattcgctgttctggatcgcgcatccaggcggcccggccatcctggaccaagtggagctcaagctgggcctgaaggaggagaagctgcgggccaccaggcatgtgctgtccgaatatgggaacatgagctccgcatgcgtcctgtttattctggacgaaatgcgcaagaagtcgatagaagaaggcaaggggaccacaggcgaagggctggaatggggcgtgctgtttggctttggcccaggactgaccgtcgaaaccgtcgtgctgcacagcctggcaacccaaagtacccactga

SEQ ID NO: 27 - DNA, 1185 bp, synthetic construct
  source 1..1185: mol_type = other DNA
atgtccaaaaccgttgaagagatctgggcagcccaacgcgctcgaggcccagctacagtgcttgcgatcggcaccgctgctcccgccaacgtggtgtaccaggcggactacccagactattatttccgcattaccaagagcgagcatatgaccgaattgaaggaaaagtttcgccggatgtgcgataagagtcagatcaccaagcgccatatgcatctgagtgaagagcttctgaaaaacaaccccgacatctgcgcgtacatggcgccctcgctcgacgcgcgtcaggacatggtggtggtggaagttccaaagctggggaaggaggctgccgcaaaagccatcaaagagtggggccggccgaagagcgccatcacccacctgattttctgcaccaccagcggcgtggacatgccgggcgccgacttccaactgactaagctgctcggcctatgcccgtcggtgcgccgcaccatgctgtaccagcaggggtgcttcgcgggcggtacagtgctgcgcctggccaaggatctggcggaaaacaatgcgggcgcccgcgtcctggtggtctgctcggaaatcaccgccgtgactttccgcggcccgtccgaaacccacctcgattcaatggttggccaggccttgtttggtgacggcgcctccgcgattatcgtgggcgccgacccggacccggtgattgagcgccctctcttccagatcgtctcggccgcccagaccattctgccggattcggacggtgcgatcgacgggcacctgcgggaggtgggcctgacctttcacctgctgaaggacgtaccgggcctgatcagcaagaacatcgagaagagcttgaaagaggccttcgccccgttaggcatcgacgattggaactcgatcttctggatcgtgcacccgggtggccctgcaatcctggatcaggtagaagccaagctccgtctgaaggtcgaaaagttgaaaaccaccaggacggtcctgtctgagtacgggaacatgagcagcgcctgtgtcttgttcatcctggatgagatgcgtcgtaacagcatggaagagggtaaagccacgactggcgaaggtctgcactggggcgtcctgttcgggttcggccccggactgacggtagagacggtcgtcctgcacagcttgcccatagcagaggcaaattga

SEQ ID NO: 28 - DNA, 1185 bp, synthetic construct
  source 1..1185: mol_type = other DNA
atggccaaggtcttgttggaggaaatccgctcctcgcagcgcgccgaaggccccgccaccatcttggccatcggcacggctaccccggcgaacgtggtgtatcaggcagactacccagactactacttccgtattaccaagagcgagcatttgaccgaccttaaagaaaaatttaagcgtatgtgcgacaagtccatgattcgcaagcgctacatgcacctgagtgaagagatcttgaaggagaatccaaacatttgtgcctacatggcccccagtctcgacgctcgccaggacgtcgtagtcgtcgaggtgccgaagctgggcaaggaggcggcggtgaaggccatcaaggaatggggccaaccgaagtcgaagatcacccacctggtattttgcacgacgtccggcgtggacatgccgggtgcggactatcagctgactaagcttctgggcctgaggccaagcgtcaacaggctgatgatgtaccagcagggctgcttcgccggcggcacagtgctacgtctcgccaaagacttggccgaaaacaatcgtggtgcgcgcgtgctggtcgtgtgtagcgagatcaccgctgtgacgtttcgcggtccatccgagagccatctggacagcctggtcggccaggcgctgttcggtgatggcgccgccgcgatcatcgtgggcgcggacccggacccggccattgagcgccccctgttccagttggtgtcggccagccagaccatccttccagactcggagggcgcgattgacggccacctgcgggaagtgggactcaccttccacttactcaaagacgtaccaggcctgatctctaagaacatccataagtccctggtggaggccttcgccccgctgggcatcagcgattggaacagtattttctggatcgcccaccctggtggtccggctatcctggaccaggtggaagccaagcttggcttggaaaaagagaagatgcgagccacccgccacgtgctgagcgaatacggcaacatgtccagcgcctgcgtgctgttcatcctcgacgagatgcgacgtcgcagcgcagaagaggggaaagccaccacaggtgagggcctcgagtggggtgtgttgttcggtttcgggccgggccttaccgtggagaccgtggtgctgcacagtcttccgataagtacccgttga

SEQ ID NO: 29 - DNA, 1185 bp, synthetic construct
  source 1..1185: mol_type = other DNA
atggccaaggtcttgttggaggaaatccgctcctcgcagcgcgccgatggccccgccaccatcttggccatcggcacggctaccccggcgaacgtggtgtatcaggcagactacccagactactacttccgtattaccaagagcgagcatttgaccgaccttaaagaaaaatttaagcgtatgtgcgacaagtccatgattcgcaagcgctacatgcacctgagtgaagagatcttgaaggagaatccaaacatttgtgcctacatggcccccagtctcgacgctcgccaggacgtcgtagtcgtcgaggtgccgaagctgggcaaggaggcggcggtgaaggccatcaaggaatggggccaaccgaagtcgaagatcacccacctggtattttgcacgacgtccggcgtggacatgccgggtgcggactatcagctgactaagcttctgggcctgaggccaagcgtcaacaggctgatgatgtaccagcagggctgcttcgccggcggcacagtgctacgtctcgccaaagacttggccgaaaacaatcgtggtgcgcgcgtgctggtcgtgtgtagcgagatcaccgctgtgacgtttcgcggtccatccgagagccatctggacagcctggtcggccaggcgctgttcggtgatggcgccgccgcgatcatcgtgggcgcggacccggacccggccattgagcgccccctgttccagttggtgtcggccagccagaccatccttccagactcggagggcgcgattgacggccacctgcgggaagtgggactcaccttccacttactcaaagacgtaccaggcctgatctctaagaacatccataagtccctggtggaggccttcgtgccgctgggcatcagcgattggaacagtattttctggatcgcccaccctggtggtccggctatcctggaccaggtggaagccaagcttggcttggaaaaagagaagatgcgagccacccgccacgtgctgagcgaatacggcaacatgtccagcgcctgcgtgctgttcatcctcgacgagatgcgacgtcgcagcgcagaagaggggaaagccaccacaggtgagggcctcgagtggggtgtgttgttcggtttcgggccgggccttaccgtggagaccgtggtgctgcacagtcttccgataagtacccgttga

SEQ ID NO: 30 - DNA, 1182 bp, synthetic construct; identical to SEQ ID NO: 22
  source 1..1182: mol_type = other DNA

SEQ ID NO: 31 - DNA, 4620 bp, synthetic construct
  source 1..4620: mol_type = other DNA
ctcgggccgtctcttgggcttgatcggccttcttgcgcatctcacgcgctcctgcggcggcctgtagggcaggctcatacccctgccgaaccgcttttgtcagccggtcggccacggcttccggcgtctcaacgcgctttgagattcccagcttttcggccaatccctgcggtgcataggcgcgtggctcgaccgcttgcgggctgatggtgacgtggcccactggtggccgctccagggcctcgtagaacgcctgaatgcgcgtgtgacgtgccttgctgccctcgatgccccgttgcagccctagatcggccacagcggccgcaaacgtggtctggtcgcgggtcatctgcgctttgttgccgatgaactccttggccgacagcctgccgtcctgcgtcagcggcaccacgaacgcggtcatgtgcgggctggtttcgtcacggtggatgctggccgtcacgatgcgatccgccccgtacttgtccgccagccacttgtgcgccttctcgaagaacgccgcctgctgttcttggctggccgacttccaccattccgggctggccgtcatgacgtactcgaccgccaacacagcgtccttgcgccgcttctctggcagcaactcgcgcagtcggcccatcgcttcatcggtgctgctggccgcccagtgctcgttctctggcgtcctgctggcgtcagcgttgggcgtctcgcgctcgcggtaggcgtgcttgagactggccgccacgttgcccattttcgccagcttcttgcatcgcatgatcgcgtatgccgccatgcctgcccctcccttttggtgtccaaccggctcgacgggggcagcgcaaggcggtgcctccggcgggccactcaatgcttgagtatactcactagactttgcttcgcaaagtcgtgaccgcctacggcggctgcggcgccctacgggcttgctctccgggcttcgccctgcgcggtcgctgcgctcccttgccagcccgtggatatgtggacgatggccgcgagcggccaccggctggctcgcttcgctcggcccgtggacaaccctgctggacaagctgatggacaggctgcgcctgcccacgagcttgaccacagggattgcccaccggctacccagccttcgaccacatacccaccggctccaactgcgcggcctgcggccttgccccatcaatttttttaattttctctggggaaaagcctccggcctgcggcctgcgcgcttcgcttgccggttggacaccaagtggaaggcgggtcaaggctcgcgcagcgaccgcgcagcggcttggccttgacgcgcctggaacgacccaagcctatgcgagtgggggcagtcgaaggcgaagcccgcccgcctgccccccgagcctcacggcggcgagtgcgggggttccaagggggcagcgccaccttgggcaaggccgaaggccgcgcagtcgatcaacaagccccggaggggccactttttgccggagggggagccgcgccgaaggcgtgggggaaccccgcaggggtgcccttctttgggcaccaaagaactagatatagggcgaaatgcgaaagacttaaaaatcaacaacttaaaaaaggggggtacgcaacagctcattgcggcaccccccgcaatagctcattgcgtaggttaaagaaaatctgtaattgactgccacttttacgcaacgcataattgttgtcgcgctgccgaaaagttgcagctgattgcgcatggtgccgcaaccgtgcggcaccctaccgcatggagataagcatggccacgcagtccagagaaatcggcattcaagccaagaacaagcccggtcactgggtgcaaacggaacgcaaagcgcatgaggcgtgggccgggcttattgcgaggaaacccacggcggcaatgctgctgcatcacctcgtggcgcagatgggccaccagaacgccgtggtggtcagccagaagacactttccaagctcatcggacgttctttgcggacggtccaatacgcagtcaaggacttggtggccgagcgctggatctccgtcgtgaagctcaacggccccggcaccgtgtcggcctacgtggtcaatgaccgcgtggcgtggggccagccccgcgaccagttgcgcctgtcggtgttcagtgccgccgtggtggttgatcacgacgaccaggacgaatcgctgttggggcatggcgacctgcgccgcatcccgaccctgtatccgggcgagcagcaactaccgaccggccccggcgaggagccgcccagccagcccggcattccgggcatggaaccagacctgccagccttgaccgaaacggaggaatgggaacggcgcgggcagcagcgcctgccgatgcccgatgagccgtgttttctggacgatggcgagccgttggagccgccgacacgggtcacgctgccgcgccggtagggcatcaaataaaacgaaaggctcagtcgaaagactgggcctttcgttttatctgttgtttgtcggtgaacgctctcctgagtaggacaaatccgccgccctagagcgcaacgcaattaatgtaagttagcgcgaattgatctggtttgacagcttatcatcgactgcacggtgcaccaatgcttctggcgtcaggcagccatcggaagctgtggtatggctgtgcaggtcgtaaatcactgcataattcgtgtcgctcaaggcgcactcccgttctggataatgttttttgcgccgacatcataacggttctggcaaatattctgaaatgagctgttgacaattaatcatccggctcgtataatgtgtggaattgtgagcggataacaattaggaggaaaaacatcttggactcctgttgatagatccagtaatgacctcagaactccatctggatttgttcagaacgctcggttgccgccgggcgttttttattggtgagaatccagattgcgttgcgctcactgcccgctttccagtcgggaaacctgtcgtgccagctgcattaatgaatcggccaacgcgcggggagaggcggtttgcgtattgggcgcatgcataaaaactgttgtaattcattaagcattctgccgacatggaagccatcacaaacggcatgatgaacctgaatcgccagcggcatcagcaccttgtcgccttgcgtataatatttgcccatgggggtgggcgaagaactccagcatgagatccccgcgctggaggatcatccagccggcgtcccggaaaacgattccgaagcccaacctttcatagaaggcggcggtggaatcgaaatctcgtgatggcaggttgggcgtcgcttggtcggtcatttcgaaccccagagtcccgctcagaagaactcgtcaagaaggcgatagaaggcgatgcgctgcgaatcgggagcggcgataccgtaaagcacgaggaagcggtcagcccattcgccgccaagctcttcagcaatatcacgggtagccaacgctatgtcctgatagcggtccgccacacccagccggccacagtcgatgaatccagaaaagcggccattttccaccatgatattcggcaagcaggcatcgccatgggtcacgacgagatcctcgccgtcgggcatgcgcgccttgagcctggcgaacagttcggctggcgcgagcccctgatgctcttcgtccagatcatcctgatcgacaagaccggcttccatccgagtacgtgctcgctcgatgcgatgtttcgcttggtggtcgaatgggcaggtagccggatcaagcgtatgcagccgccgcattgcatcagccatgatggatactttctcggcaggagcaaggtgagatgacaggagatcctgccccggcacttcgcccaatagcagccagtcccttcccgcttcagtgacaacgtcgagcacagctgcgcaaggaacgcccgtcgtggccagccacgatagccgcgctgcctcgtcctgcagttcattcagggcaccggacaggtcggtcttgacaaaaagaaccgggcgcccctgcgctgacagccggaacacggcggcatcagagcagccgattgtctgttgtgcccagtcatagccgaatagcctctccacccaagcggccggagaacctgcgtgcaatccatcttgttcaatcatgcgaaacgatcctcatcctgtctcttgatcagatcttgatcccctgcgccatcagatccttggcggcaagaaagccatccagtttactttgcagggcttcccaaccttaccagagggcgccccagctggcaattccggttcgcttgctgtccataaaaccgcccagtctagctatcgccatgtaagcccactgcaagctacctgctttctctttgcgcttgcgttttcccttgtccagatagcccagtagctgacattcatcccaggtggcacttttcggggaaatgtgcgcgcccgcgttcctgctggcgctgggcctgtttctggcgctggacttcccgctgttccgtcagcagcttttcgcccacggccttgatgatcgcggcggccttggcctgcatatcccgattcaacggccccagggcgtccagaacgggcttcaggcgctcccgaaggt

SEQ ID NO: 32 - DNA, 5775 bp, synthetic construct
  source 1..5775: mol_type = other DNA
ctcgggccgtctcttgggcttgatcggccttcttgcgcatctcacgcgctcctgcggcggcctgtagggcaggctcatacccctgccgaaccgcttttgtcagccggtcggccacggcttccggcgtctcaacgcgctttgagattcccagcttttcggccaatccctgcggtgcataggcgcgtggctcgaccgcttgcgggctgatggtgacgtggcccactggtggccgctccagggcctcgtagaacgcctgaatgcgcgtgtgacgtgccttgctgccctcgatgccccgttgcagccctagatcggccacagcggccgcaaacgtggtctggtcgcgggtcatctgcgctttgttgccgatgaactccttggccgacagcctgccgtcctgcgtcagcggcaccacgaacgcggtcatgtgcgggctggtttcgtcacggtggatgctggccgtcacgatgcgatccgccccgtacttgtccgccagccacttgtgcgccttctcgaagaacgccgcctgctgttcttggctggccgacttccaccattccgggctggccgtcatgacgtactcgaccgccaacacagcgtccttgcgccgcttctctggcagcaactcgcgcagtcggcccatcgcttcatcggtgctgctggccgcccagtgctcgttctctggcgtcctgctggcgtcagcgttgggcgtctcgcgctcgcggtaggcgtgcttgagactggccgccacgttgcccattttcgccagcttcttgcatcgcatgatcgcgtatgccgccatgcctgcccctcccttttggtgtccaaccggctcgacgggggcagcgcaaggcggtgcctccggcgggccactcaatgcttgagtatactcactagactttgcttcgcaaagtcgtgaccgcctacggcggctgcggcgccctacgggcttgctctccgggcttcgccctgcgcggtcgctgcgctcccttgccagcccgtggatatgtggacgatggccgcgagcggccaccggctggctcgcttcgctcggcccgtggacaaccctgctggacaagctgatggacaggctgcgcctgcccacgagcttgaccacagggattgcccaccggctacccagccttcgaccacatacccaccggctccaactgcgcggcctgcggccttgccccatcaatttttttaattttctctggggaaaagcctccggcctgcggcctgcgcgcttcgcttgccggttggacaccaagtggaaggcgggtcaaggctcgcgcagcgaccgcgcagcggcttggccttgacgcgcctggaacgacccaagcctatgcgagtgggggcagtcgaaggcgaagcccgcccgcctgccccccgagcctcacggcggcgagtgcgggggttccaagggggcagcgccaccttgggcaaggccgaaggccgcgcagtcgatcaacaagccccggaggggccactttttgccggagggggagccgcgccgaaggcgtgggggaaccccgcaggggtgcccttctttgggcaccaaagaactagatatagggcgaaatgcgaaagacttaaaaatcaacaacttaaaaaaggggggtacgcaacagctcattgcggcaccccccgcaatagctcattgcgtaggttaaagaaaatctgtaattgactgccacttttacgcaacgcataattgttgtcgcgctgccgaaaagttgcagctgattgcgcatggtgccgcaaccgtgcggcaccctaccgcatggagataagcatggccacgcagtccagagaaatcggcattcaagccaagaacaagcccggtcactgggtgcaaacggaacgcaaagcgcatgaggcgtgggccgggcttattgcgaggaaacccacggcggcaatgctgctgcatcacctcgtggcgcagatgggccaccagaacgccgtggtggtcagccagaagacactttccaagctcatcggacgttctttgcggacggtccaatacgcagtcaaggacttggtggccgagcgctggatctccgtcgtgaagctcaacggccccggcaccgtgtcggcctacgtggtcaatgaccgcgtggcgtggggccagccccgcgaccagttgcgcctgtcggtgttcagtgccgccgtggtggttgatcacgacgaccaggacgaatcgctgttggggcatggcgacctgcgccgcatcccgaccctgtatccgggcgagcagcaactaccgaccggccccggcgaggagccgcccagccagcccggcattccgggcatggaaccagacctgccagccttgaccgaaacggaggaatgggaacggcgcgggcagcagcgcctgccgatgcccgatgagccgtgttttctggacgatggcgagccgttggagccgccgacacgggtcacgctgccgcgccggtagggcatcaaataaaacgaaaggctcagtcgaaagactgggcctttcgttttatctgttgtttgtcggtgaacgctctcctgagtaggacaaatccgccgccctagagcgcaacgcaattaatgtaagttagcgcgaattgatctggtttgacagcttatcatcgactgcacggtgcaccaatgcttctggcgtcaggcagccatcggaagctgtggtatggctgtgcaggtcgtaaatcactgcataattcgtgtcgctcaaggcgcactcccgttctggataatgttttttgcgccgacatcataacggttctggcaaatattctgaaatgagctgttgacaattaatcatccggctcgtataatgtgtggaattgtgagcggataacaattaggaggaaaaacatatggcaactgaggagatgaagaaattggccaccgtgatggccattggcacggccaaccctccgaactgctactaccaggccgactttcccgacttctacttccgcgtcaccaacagcgaccacctcatcaacctcaagcaaaagttcaagcgcctttgtgaaaactcaaggattgagaagcgttaccttcatgtgaccgaagagattctcaaggaaaacccaaacattgctgcctacgaggcaacctcgttgaatgtaagacacaaaatgcaagtgaaaggagttgcagagcttgggaaagaggctgccctcaaggccatcaaagaatggggccaacccaagtccaagatcacacatctcatcgtgtgttgcctagccggcgttgacatgcccggcgcggattatcaactcactaagcttcttgaccttgacccttccgtcaagcgttttatgttttaccacctaggatgctacgctggtggcactgtccttcgccttgcaaaggacatagcggagaacaacaagggagctcgtgttctcatcgtttgctcagagatgacaacaacttgttttcgtgggccatctgaaacccatctggactccatgataggccaagcaatattaggcgatggggctgcagctgtcatagttggcgcagatccagacctaaccgttgagaggcccatattcgagttggtttccacagcccagactattgtacccgaatcccatggtgcaattgagggccacttgcttgaatctggactcagtttccatttgtacaagaccgttcctacactaatctctaacaacattaaaacttgcctttctgatgctttcactcctctaaacattagcgattggaactctcttttctggatcgcacaccctggtggtcctgccatcctagaccaagttactgctaaggttggtcttgaaaaggagaaactcaaggtaactagacaagtgttgaaggactatggaaacatgtcgagtgctacggtgtttttcatcatggatgagatgaggaagaagtcactcgaaaacggtcaagcaaccactggagaagggctcgagtggggtgttttgtttgggttcgggcctggaatcaccgttgaaactgtagtgctacgcagtgtgcccgtaattagctagcttggactcctgttgatagatccagtaatgacctcagaactccatctggatttgttcagaacgctcggttgccgccgggcgttttttattggtgagaatccagattgcgttgcgctcactgcccgctttccagtcgggaaacctgtcgtgccagctgcattaatgaatcggccaacgcgcggggagaggcggtttgcgtattgggcgcatgcataaaaactgttgtaattcattaagcattctgccgacatggaagccatcacaaacggcatgatgaacctgaatcgccagcggcatcagcaccttgtcgccttgcgtataatatttgcccatgggggtgggcgaagaactccagcatgagatccccgcgctggaggatcatccagccggcgtcccggaaaacgattccgaagcccaacctttcatagaaggcggcggtggaatcgaaatctcgtgatggcaggttgggcgtcgcttggtcggtcatttcgaaccccagagtcccgctcagaagaactcgtcaagaaggcgatagaaggcgatgcgctgcgaatcgggagcggcgataccgtaaagcacgaggaagcggtcagcccattcgccgccaagctcttcagcaatatcacgggtagccaacgctatgtcctgatagcggtccgccacacccagccggccacagtcgatgaatccagaaaagcggccattttccaccatgatattcggcaagcaggcatcgccatgggtcacgacgagatcctcgccgtcgggcatgcgcgccttgagcctggcgaacagttcggctggcgcgagcccctgatgctcttcgtccagatcatcctgatcgacaagaccggcttccatccgagtacgtgctcgctcgatgcgatgtttcgcttggtggtcgaatgggcaggtagccggatcaagcgtatgcagccgccgcattgcatcagccatgatggatactttctcggcaggagcaaggtgagatgacaggagatcctgccccggcacttcgcccaatagcagccagtcccttcccgcttcagtgacaacgtcgagcacagctgcgcaaggaacgcccgtcgtggccagccacgatagccgcgctgcctcgtcctgcagttcattcagggcaccggacaggtcggtcttgacaaaaagaaccgggcgcccctgcgctgacagccggaacacggcggcatcagagcagccgattgtctgttgtgcccagtcatagccgaatagcctctccacccaagcggccggagaacctgcgtgcaatccatcttgttcaatcatgcgaaacgatcctcatcctgtctcttgatcagatcttgatcccctgcgccatcagatccttggcggcaagaaagccatccagtttactttgcagggcttcccaaccttaccagagggcgccccagctggcaattccggttcgcttgctgtccataaaaccgcccagtctagctatcgccatgtaagcccactgcaagctacctgctttctctttgcgcttgcgttttcccttgtccagatagcccagtagctgacattcatcccaggtggcacttttcggggaaatgtgcgcgcccgcgttcctgctggcgctgggcctgtttctggcgctggacttcccgctgttccgtcagcagcttttcgcccacggccttgatgatcgcggcggccttggcctgcatatcccgattcaacggccccagggcgtccagaacgggcttcaggcgctcccgaaggt

SEQ ID NO: 33 - DNA, 4457 bp, synthetic construct
  source 1..4457: mol_type = other DNA
ctcgggccgtctcttgggcttgatcggccttcttgcgcatctcacgcgctcctgcggcggcctgtagggcaggctcatacccctgccgaaccgcttttgtcagccggtcggccacggcttccggcgtctcaacgcgctttgagattcccagcttttcggccaatccctgcggtgcataggcgcgtggctcgaccgcttgcgggctgatggtgacgtggcccactggtggccgctccagggcctcgtagaacgcctgaatgcgcgtgtgacgtgccttgctgccctcgatgccccgttgcagccctagatcggccacagcggccgcaaacgtggtctggtcgcgggtcatctgcgctttgttgccgatgaactccttggccgacagcctgccgtcctgcgtcagcggcaccacgaacgcggtcatgtgcgggctggtttcgtcacggtggatgctggccgtcacgatgcgatccgccccgtacttgtccgccagccacttgtgcgccttctcgaagaacgccgcctgctgttcttggctggccgacttccaccattccgggctggccgtcatgacgtactcgaccgccaacacagcgtccttgcgccgcttctctggcagcaactcgcgcagtcggcccatcgcttcatcggtgctgctggccgcccagtgctcgttctctggcgtcctgctggcgtcagcgttgggcgtctcgcgctcgcggtaggcgtgcttgagactggccgccacgttgcccattttcgccagcttcttgcatcgcatgatcgcgtatgccgccatgcctgcccctcccttttggtgtccaaccggctcgacgggggcagcgcaaggcggtgcctccggcgggccactcaatgcttgagtatactcactagactttgcttcgcaaagtcgtgaccgcctacggcggctgcggcgccctacgggcttgctctccgggcttcgccctgcgcggtcgctgcgctcccttgccagcccgtggatatgtggacgatggccgcgagcggccaccggctggctcgcttcgctcggcccgtggacaaccctgctggacaagctgatggacaggctgcgcctgcccacgagcttgaccacagggattgcccaccggctacccagccttcgaccacatacccaccggctccaactgcgcggcctgcggccttgccccatcaatttttttaattttctctggggaaaagcctccggcctgcggcctgcgcgcttcgcttgccggttggacaccaagtggaaggcgggtcaaggctcgcgcagcgaccgcgcagcggcttggccttgacgcgcctggaacgacccaagcctatgcgagtgggggcagtcgaaggcgaagcccgcccgcctgccccccgagcctcacggcggcgagtgcgggggttccaagggggcagcgccaccttgggcaaggccgaaggccgcgcagtcgatcaacaagccccggaggggccactttttgccggagggggagccgcgccgaaggcgtgggggaaccccgcaggggtgcccttctttgggcaccaaagaactagatatagggcgaaatgcgaaagacttaaaaatcaacaacttaaaaaaggggggtacgcaacagctcattgcggcaccccccgcaatagctcattgcgtaggttaaagaaaatctgtaattgactgccacttttacgcaacgcataattgttgtcgcgctgccgaaaagttgcagctgattgcgcatggtgccgcaaccgtgcggcaccctaccgcatggagataagcatggccacgcagtccagagaaatcggcattcaagccaagaacaagcccggtcactgggtgcaaacggaacgcaaagcgcatgaggcgtgggccgggcttattgcgaggaaacccacggcggcaatgctgctgcatcacctcgtggcgcagatgggccaccagaacgccgtggtggtcagccagaagacactttccaagctcatcggacgttctttgcggacggtccaatacgcagtcaaggacttggtggccgagcgctggatctccgtcgtgaagctcaacggccccggcaccgtgtcggcctacgtggtcaatgaccgcgtggcgtggggccagccccgcgaccagttgcgcctgtcggtgttcagtgccgccgtggtggttgatcacgacgaccaggacgaatcgctgttggggcatggcgacctgcgccgcatcccgaccctgtatccgggcgagcagcaactaccgaccggccccggcgaggagccgcccagccagcccggcattccgggcatggaaccagacctgccagccttgaccgaaacggaggaatgggaacggcgcgggcagcagcgcctgccgatgcccgatgagccgtgttttctggacgatggcgagccgttggagccgccgacacgggtcacgctgccgcgccggtagggcatcaaataaaacgaaaggctcagtcgaaagactgggcctttcgttttatctgttgtttgtcggtgaacgctctcctgagtaggacaaatccgccgccctagattaattaagcccattgacaaggctctcgcggccaggtataattgcacgacctagggcccaagttcacttaaaaaggagatcaacaatgaaagcaattttcgtactgaaacatcttaatcatgctaacgagattttctacttggactcctgttgatagatccagtaatgacctcagaactccatctggatttgttcagaacgctcggttgccgccgggcgttttttattggtgagaatccagattgcgttgcgctcactgcccgctttccagtcgggaaacctgtcgtgccagctgcattaatgaatcggccaacgcgcggggagaggcggtttgcgtattgggcgcatgcataaaaactgttgtaattcattaagcattctgccgacatggaagccatcacaaacggcatgatgaacctgaatcgccagcggcatcagcaccttgtcgccttgcgtataatatttgcccatgggggtgggcgaagaactccagcatgagatccccgcgctggaggatcatccagccggcgtcccggaaaacgattccgaagcccaacctttcatagaaggcggcggtggaatcgaaatctcgtgatggcaggttgggcgtcgcttggtcggtcatttcgaaccccagagtcccgctcagaagaactcgtcaagaaggcgatagaaggcgatgcgctgcgaatcgggagcggcgataccgtaaagcacgaggaagcggtcagcccattcgccgccaagctcttcagcaatatcacgggtagccaacgctatgtcctgatagcggtccgccacacccagccggccacagtcgatgaatccagaaaagcggccattttccaccatgatattcggcaagcaggcatcgccatgggtcacgacgagatcctcgccgtcgggcatgcgcgccttgagcctggcgaacagttcggctggcgcgagcccctgatgctcttcgtccagatcatcctgatcgacaagaccggcttccatccgagtacgtgctcgctcgatgcgatgtttcgcttggtggtcgaatgggcaggtagccggatcaagcgtatgcagccgccgcattgcatcagccatgatggatactttctcggcaggagcaaggtgagatgacaggagatcctgccccggcacttcgcccaatagcagccagtcccttcccgcttcagtgacaacgtcgagcacagctgcgcaaggaacgcccgtcgtggccagccacgatagccgcgctgcctcgtcctgcagttcattcagggcaccggacaggtcggtcttgacaaaaagaaccgggcgcccctgcgctgacagccggaacacggcggcatcagagcagccgattgtctgttgtgcccagtcatagccgaatagcctctccacccaagcggccggagaacctgcgtgcaatccatcttgttcaatcatgcgaaacgatcctcatcctgtctcttgatcagatcttgatcccctgcgccatcagatccttggcggcaagaaagccatccagtttactttgcagggcttcccaaccttaccagagggcgccccagctggcaattccggttcgcttgctgtccataaaaccgcccagtctagctatcgccatgtaagcccactgcaagctacctgctttctctttgcgcttgcgttttcccttgtccagatagcccagtagctgacattcatcccaggtggcacttttcggggaaatgtgcgcgcccgcgttcctgctggcgctgggcctgtttctggcgctggacttcccgctgttccgtcagcagcttttcgcccacggccttgatgatcgcggcggccttggcctgcatatcccgattcaacggccccagggcgtccagaacgggcttcaggcgctcccgaaggt

SEQ ID NO: 34 - DNA, 5642 bp, synthetic construct
  source 1..5642: mol_type = other DNA
ctcgggccgtctcttgggcttgatcggccttcttgcgcatctcacgcgctcctgcggcggcctgtagggcaggctcatacccctgccgaaccgcttttgtcagccggtcggccacggcttccggcgtctcaacgcgctttgagattcccagcttttcggccaatccctgcggtgcataggcgcgtggctcgaccgcttgcgggctgatggtgacgtggcccactggtggccgctccagggcctcgtagaacgcctgaatgcgcgtgtgacgtgccttgctgccctcgatgccccgttgcagccctagatcggccacagcggccgcaaacgtggtctggtcgcgggtcatctgcgctttgttgccgatgaactccttggccgacagcctgccgtcctgcgtcagcggcaccacgaacgcggtcatgtgcgggctggtttcgtcacggtggatgctggccgtcacgatgcgatccgccccgtacttgtccgccagccacttgtgcgccttctcgaagaacgccgcctgctgttcttggctggccgacttccaccattccgggctggccgtcatgacgtactcgaccgccaacacagcgtccttgcgccgcttctctggcagcaactcgcgcagtcggcccatcgcttcatcggtgctgctggccgcccagtgctcgttctctggcgtcctgctggcgtcagcgttgggcgtctcgcgctcgcggtaggcgtgcttgagactggccgccacgttgcccattttcgccagcttcttgcatcgcatgatcgcgtatgccgccatgcctgcccctcccttttggtgtccaaccggctcgacgggggcagcgcaaggcggtgcctccggcgggccactcaatgcttgagtatactcactagactttgcttcgcaaagtcgtgaccgcctacggcggctgcggcgccctacgggcttgctctccgggcttcgccctgcgcggtcgctgcgctcccttgccagcccgtggatatgtggacgatggccgcgagcggccaccggctggctcgcttcgctcggcccgtggacaaccctgctggacaagctgatggacaggctgcgcctgcccacgagcttgaccacagggattgcccaccggctacccagccttcgaccacatacccaccggctccaactgcgcggcctgcggccttgccccatcaatttttttaattttctctggggaaaagcctccggcctgcggcctgcgcgcttcgcttgccggttggacaccaagtggaaggcgggtcaaggctcgcgcagcgaccgcgcagcggcttggccttgacgcgcctggaacgacccaagcctatgcgagtgggggcagtcgaaggcgaagcccgcccgcctgccccccgagcctcacggcggcgagtgcgggggttccaagggggcagcgccaccttgggcaaggccgaaggccgcgcagtcgatcaacaagccccggaggggccactttttgccggagggggagccgcgccgaaggcgtgggggaaccccgcaggggtgcccttctttgggcaccaaagaactagatatagggcgaaatgcgaaagacttaaaaatcaacaacttaaaaaaggggggtacgcaacagctcattgcggcaccccccgcaatagctcattgcgtaggttaaagaaaatctgtaattgactgccacttttacgcaacgcataattgttgtcgcgctgccgaaaagttgcagctgattgcgcatggtgccgcaaccgtgcggcaccctaccgcatggagataagcatggccacgcagtccagagaaatcggcattcaagccaagaacaagcccggtcactgggtgcaaacggaacgcaaagcgcatgaggcgtgggccgggcttattgcgaggaaacccacggcggcaatgctgctgcatcacctcgtggcgcagatgggccaccagaacgccgtggtggtcagccagaagacactttccaagctcatcggacgttctttgcggacggtccaatacgcagtcaaggacttggtggccgagcgctggatctccgtcgtgaagctcaacggccccggcaccgtgtcggcctacgtggtcaatgaccgcgtggcgtggggccagccccgcgaccagttgcgcctgtcggtgttcagtgccgccgtggtggttgatcacgacgaccaggacgaatcgctgttggggcatggcgacctgcgccgcatcccgaccctgtatccgggcgagcagcaactaccgaccggccccggcgaggagccgcccagccagcccggcattccgggcatggaaccagacctgccagccttgaccgaaacggaggaatgggaacggcgcgggcagcagcgcctgccgatgcccgatgagccgtgttttctggacgatggcgagccgttggagccgccgacacgggtcacgctgccgcgccggtagggcatcaaataaaacgaaaggctcagtcgaaagactgggcctttcgttttatctgttgtttgtcggtgaacgctctcctgagtaggacaaatccgccgccctagattaattaagcccattgacaaggctctcgcggccaggtataattgcacgacctagggcccaagttcacttaaaaaggagatcaacaatgaaagcaattttcgtactgaaacatcttaatcatgctaacgagattttctaatgtccaaaaccgttgaagagatctgggcagcccaacgcgctcgaggcccagctacagtgcttgcgatcggcaccgctgctcccgccaacgtggtgtaccaggcggactacccagactattatttccgcattaccaagagcgagcatatgaccgaattgaaggaaaagtttcgccggatgtgcgataagagtatgatcaccaagcgccatatgcatctgagtgaagagcttctgaaaaacaaccccgacatctgcgcgtacatggcgccctcgctcgacgcgcgtcaggacatggtggtggtggaagttccaaagctggggaaggaggctgccgcaaaagccatcaaagagtggggccggccgaagagcgccatcacccacctgattttctgcaccaccagcggcgtggacatgccgggcgccgacttccaactgactaagctgctcggcctatgcccgtcggtgcgccgcaccatgctgtaccagcaggggtgcttcgcgggcggtacagtgctgcgcctggccaaggatctggcggaaaacaatgcgggcgcccgcgtcctggtggtctgctcggaaatcaccgccgtgactttccgcggcccgtccgaaacccacctcgattcaatggttggccaggccttgtttggtgacggcgcctccgcgattatcgtgggcgccgacccggacccggtgattgagcgccctctcttccagatcgtctcggccgcccagaccattctgccggattcggacggtgcgatcgacgggcacctgcgggaggtgggcctgacctttcacctgctgaaggacgtaccgggcctgatcagcaagaacatcgagaagagcttgaaagaggccttcgccccgttaggcatcgacgattggaactcgatcttctggatcgtgcacccgggtggccctgcaatcctggatcaggtagaagccaagctccgtctgaaggtcgaaaagttgaaaaccaccaggacggtcctgtctgagtacgggaacatgagcagcgcctgtgtcttgttcatcctggatgagatgcgtcgtaacagcatggaagagggtaaagccacgactggcgaaggtctgcactggggcgtcctgttcgggttcggccccggactgacggtagagacggtcgtcctgcacagcttgcccatagcagaggcaaattgacttggactcctgttgatagatccagtaatgacctcagaactccatctggatttgttcagaacgctcggttgccgccgggcgttttttattggtgagaatccagattgcgttgcgctcactgcccgctttccagtcgggaaacctgtcgtgccagctgcattaatgaatcggccaacgcgcggggagaggcggtttgcgtattgggcgcatgcataaaaactgttgtaattcattaagcattctgccgacatggaagccatcacaaacggcatgatgaacctgaatcgccagcggcatcagcaccttgtcgccttgcgtataatatttgcccatgggggtgggcgaagaactccagcatgagatccccgcgctggaggatcatccagccggcgtcccggaaaacgattccgaagcccaacctttcatagaaggcggcggtggaatcgaaatctcgtgatggcaggttgggcgtcgcttggtcggtcatttcgaaccccagagtcccgctcagaagaactcgtcaagaaggcgatagaaggcgatgcgctgcgaatcgggagcggcgataccgtaaagcacgaggaagcggtcagcccattcgccgccaagctcttcagcaatatcacgggtagccaacgctatgtcctgatagcggtccgccacacccagccggccacagtcgatgaatccagaaaagcggccattttccaccatgatattcggcaagcaggcatcgccatgggtcacgacgagatcctcgccgtcgggcatgcgcgccttgagcctggcgaacagttcggctggcgcgagcccctgatgctcttcgtccagatcatcctgatcgacaagaccggcttccatccgagtacgtgctcgctcgatgcgatgtttcgcttggtggtcgaatgggcaggtagccggatcaagcgtatgcagccgccgcattgcatcagccatgatggatactttctcggcaggagcaaggtgagatgacaggagatcctgccccggcacttcgcccaatagcagccagtcccttcccgcttcagtgacaacgtcgagcacagctgcgcaaggaacgcccgtcgtggccagccacgatagccgcgctgcctcgtcctgcagttcattcagggcaccggacaggtcggtcttgacaaaaagaaccgggcgcccctgcgctgacagccggaacacggcggcatcagagcagccgattgtctgttgtgcccagtcatagccgaatagcctctccacccaagcggccggagaacctgcgtgcaatccatcttgttcaatcatgcgaaacgatcctcatcctgtctcttgatcagatcttgatcccctgcgccatcagatccttggcggcaagaaagccatccagtttactttgcagggcttcccaaccttaccagagggcgccccagctggcaattccggttcgcttgctgtccataaaaccgcccagtctagctatcgccatgtaagcccactgcaagctacctgctttctctttgcgcttgcgttttcccttgtccagatagcccagtagctgacattcatcccaggtggcacttttcggggaaatgtgcgcgcccgcgttcctgctggcgctgggcctgtttctggcgctggacttcccgctgttccgtcagcagcttttcgcccacggccttgatgatcgcggcggccttggcctgcatatcccgattcaacggccccagggcgtccagaacgggcttcaggcgctcccgaaggt

SEQ ID NO: 35 - DNA, 5642 bp, synthetic construct
  source 1..5642: mol_type = other DNA
ctcgggccgtctcttgggcttgatcggccttcttgcgcatctcacgcgctcctgcggcggcctgtagggcaggctcatacccctgccgaaccgcttttgtcagccggtcggccacggcttccggcgtctcaacgcgctttgagattcccagcttttcggccaatccctgcggtgcataggcgcgtggctcgaccgcttgcgggctgatggtgacgtggcccactggtggccgctccagggcctcgtagaacgcctgaatgcgcgtgtgacgtgccttgctgccctcgatgccccgttgcagccctagatcggccacagcggccgcaaacgtggtctggtcgcgggtcatctgcgctttgttgccgatgaactccttggccgacagcctgccgtcctgcgtcagcggcaccacgaacgcggtcatgtgcgggctggtttcgtcacggtggatgctggccgtcacgatgcgatccgccccgtacttgtccgccagccacttgtgcgccttctcgaagaacgccgcctgctgttcttggctggccgacttccaccattccgggctggccgtcatgacgtactcgaccgccaacacagcgtccttgcgccgcttctctggcagcaactcgcgcagtcggcccatcgcttcatcggtgctgctggccgcccagtgctcgttctctggcgtcctgctggcgtcagcgttgggcgtctcgcgctcgcggtaggcgtgcttgagactggccgccacgttgcccattttcgccagcttcttgcatcgcatgatcgcgtatgccgccatgcctgcccctcccttttggtgtccaaccggctcgacgggggcagcgcaaggcggtgcctccggcgggccactcaatgcttgagtatactcactagactttgcttcgcaaagtcgtgaccgcctacggcggctgcggcgccctacgggcttgctctccgggcttcgccctgcgcggtcgctgcgctcccttgccagcccgtggatatgtggacgatggccgcgagcggccaccggctggctcgcttcgctcggcccgtggacaaccctgctggacaagctgatggacaggctgcgcctgcccacgagcttgaccacagggattgcccaccggctacccagccttcgaccacatacccaccggctccaactgcgcggcctgcggccttgccccatcaatttttttaattttctctggggaaaagcctccggcctgcggcctgcgcgcttcgcttgccggttggacaccaagtggaaggcgggtcaaggctcgcgcagcgaccgcgcagcggcttggccttgacgcgcctggaacgacccaagcctatgcgagtgggggcagtcgaaggcgaagcccgcccgcctgccccccgagcctcacggcggcgagtgcgggggttccaagggggcagcgccaccttgggcaaggccgaaggccgcgcagtcgatcaacaagccccggaggggccactttttgccggagggggagccgcgccgaaggcgtgggggaaccccgcaggggtgcccttctttgggcaccaaagaactagatatagggcgaaatgcgaaagacttaaaaatcaacaacttaaaaaaggggggtacgcaacagctcattgcggcaccccccgcaatagctcattgcgtaggttaaagaaaatctgtaattgactgccacttttacgcaacgcataattgttgtcgcgctgccgaaaagttgcagctgattgcgcatggtgccgcaaccgtgcggcaccctaccgcatggagataagcatggccacgcagtccagagaaatcggcattcaagccaagaacaagcccggtcactgggtgcaaacggaacgcaaagcgcatgaggcgtgggccgggcttattgcgaggaaacccacggcggcaatgctgctgcatcacctcgtggcgcagatgggccaccagaacgccgtggtggtcagccagaagacactttccaagctcatcggacgttctttgcggacggtccaatacgcagtcaaggacttggtggccgagcgctggatctccgtcgtgaagctcaacggccccggcaccgtgtcggcctacgtggtcaatgaccgcgtggcgtggggccagccccgcgaccagttgcgcctgtcggtgttcagtgccgccgtggtggttgatcacgacgaccaggacgaatcgctgttggggcatggcgacctgcgccgcatcccgaccctgtatccgggcgagcagcaactaccgaccggccccggcgaggagccgcccagccagcccggcattccgggcatggaaccagacctgccagccttgaccgaaacggaggaatgggaacggcgcgggcagcagcgcctgccgatgcccgatgagccgtgttttctggacgatggcgagccgttggagccgccgacacgggtcacgctgccgcgccggtagggcatcaaataaaacgaaaggctcagtcgaaagactgggcctttcgttttatctgttgtttgtcggtgaacgctctcctgagtaggacaaatccgccgccctagattaattaagcccattgacaaggctctcgcggccaggtataattgcacgacctagggtccaagttcacttaaaaaggagatcaacaatgaaagcaattttcgtactgaaacatcttaatcatgctaacgagattttctaatgtccaaaaccgttgaagagatctgggcagcccaacgcgctcgaggcccagctacagtgcttgcgatcggcaccgctgctcccgccaacgtggtgtaccaggcggactacgcagactattatttccgcattaccaagagcgagcatatgaccgaattgaaggaaaagtttcgccggatgtgcgataagagtatgatcaccaagcgccatatgcatctgagtgaagagcttctgaaaaacaaccccgacatctgcgcgtacatggcgccctcgctcgacgcgcgtcaggacatggtggtggtggaagttccaaagctggggaaggaggctgccgcaaaagccatcaaagagtggggccggccgaagagcgccatcacccacctgattttctgcaccaccagcggcgtggacatgccgggcgccgacttccaactgactaagctgctcggcctatgcccgtcggtgcgccgcaccatgctgtaccagcaggggtgcttcgcgggcggtacagtgctgcgcctggccaaggatctggcggaaaacaatgcgggcgcccgcgtcctggtggtctgctcggaaatcaccgccgtgactttccgcggcccgtccgaaacccacctcgattcaatggttggccaggccttgtttggtgacggcgcctccgcgattatcgtgggcgccgacccggacccggtgattgagcgccctctcttccagatcgtctcggccgcccagaccattctgccggattcggacggtgcgatcgacgggcacctgcgggaggtgggcctgacctttcacctgctgaaggacgtaccgggcctgatcagcaagaacatcgagaagagcttgaaagaggccttcgccccgttaggcatcgacgattggaactcgatcttctggatcgtgcacccgggtggccctgcaatcctggatcaggtagaagccaagctccgtctgaaggtcgaaaagttgaaaaccaccaggacggtcctgtctgagtacgggaacatgagcagcgcctgtgtcttgttcatcctggatgagatgcgtcgtaacagcatggaagagggtaaagccacgactggcgaaggtctgcactggggcgtcctgttcgggttcggccccggactgacggtagagacggtcgtcctgcacagcttgcccatagcagaggcaaattgacttggactcctgttgatagatccagtaatgacctcagaactccatctggatttgttcagaacgctcggttgccgccgggcgttttttattggtgagaatccagattgcgttgcgctcactgcccgctttccagtcgggaaacctgtcgtgccagctgcattaatgaatcggccaacgcgcggggagaggcggtttgcgtattgggcgcatgcataaaaactgttgtaattcattaagcattctgccgacatggaagccatcacaaacggcatgatgaacctgaatcgccagcggcatcagcaccttgtcgccttgcgtataatatttgcccatgggggtgggcgaagaactccagcatgagatccccgcgctggaggatcatccagccggcgtcccggaaaacgattccgaagcccaacctttcatagaaggcggcggtggaatcgaaatctcgtgatggcaggttgggcgtcgcttggtcggtcatttcgaaccccagagtcccgctcagaagaactcgtcaagaaggcgatagaaggcgatgcgctgcgaatcgggagcggcgataccgtaaagcacgaggaagcggtcagcccattcgccgccaagctcttcagcaatatcacgggtagccaacgctatgtcctgatagcggtccgccacacccagccggccacagtcgatgaatccagaaaagcggccattttccaccatgatattcggcaagcaggcatcgccatgggtcacgacgagatcctcgccgtcgggcatgcgcgccttgagcctggcgaacagttcggctggcgcgagcccctgatgctcttcgtccagatcatcctgatcgacaagaccggcttccatccgagtacgtgctcgctcgatgcgatgtttcgcttggtggtcgaatgggcaggtagccggatcaagcgtatgcagccgccgcattgcatcagccatgatggatactttctcggcaggagcaaggtgagatgacaggagatcctgccccggcacttcgcccaatagcagccagtcccttcccgcttcagtgacaacgtcgagcacagctgcgcaaggaacgcccgtcgtggccagccacgatagccgcgctgcctcgtcctgcagttcattcagggcaccggacaggtcggtcttgacaaaaagaaccgggcgcccctgcgctgacagccggaacacggcggcatcagagcagccgattgtctgttgtgcccagtcatagccgaatagcctctccacccaagcggccggagaacctgcgtgcaatccatcttgttcaatcatgcgaaacgatcctcatcctgtctcttgatcagatcttgatcccctgcgccatcagatccttggcggcaagaaagccatccagtttactttgcagggcttcccaaccttaccagagggcgccccagctggcaattccggttcgcttgctgtccataaaaccgcccagtctagctatcgccatgtaagcccactgcaagctacctgctttctctttgcgcttgcgttttcccttgtccagatagcccagtagctgacattcatcccaggtggcacttttcggggaaatgtgcgcgcccgcgttcctgctggcgctgggcctgtttctggcgctggacttcccgctgttccgtcagcagcttttcgcccacggccttgatgatcgcggcggccttggcctgcatatcccgattcaacggccccagggcgtccagaacgggcttcaggcgctcccgaaggt

SEQ ID NO: 36 - DNA, 5642 bp, synthetic construct
  source 1..5642: mol_type = other DNA
ctcgggccgtctcttgggcttgatcggccttcttgcgcatctcacgcgctcctgcggcggcctgtagggcaggctcatacccctgccgaaccgcttttgtcagccggtcggccacggcttccggcgtctcaacgcgctttgagattcccagcttttcggccaatccctgcggtgcataggcgcgtggctcgaccgcttgcgggctgatggtgacgtggcccactggtggccgctccagggcctcgtagaacgcctgaatgcgcgtgtgacgtgccttgctgccctcgatgccccgttgcagccctagatcggccacagcggccgcaaacgtggtctggtcgcgggtcatctgcgctttgttgccgatgaactccttggccgacagcctgccgtcctgcgtcagcggcaccacgaacgcggtcatgtgcgggctggtttcgtcacggtggatgctggccgtcacgatgcgatccgccccgtacttgtccgccagccacttgtgcgccttctcgaagaacgccgcctgctgttcttggctggccgacttccaccattccgggctggccgtcatgacgtactcgaccgccaacacagcgtccttgcgccgcttctctggcagcaactcgcgcagtcggcccatcgcttcatcggtgctgctggccgcccagtgctcgttctctggcgtcctgctggcgtcagcgttgggcgtctcgcgctcgcggtaggcgtgcttgagactggccgccacgttgcccattttcgccagcttcttgcatcgcatgatcgcgtatgccgccatgcctgcccctcccttttggtgtccaaccggctcgacgggggcagcgcaaggcggtgcctccggcgggccactcaatgcttgagtatactcactagactttgcttcgcaaagtcgtgaccgcctacggcggctgcggcgccctacgggcttgctctccgggcttcgccctgcgcggtcgctgcgctcccttgccagcccgtggatatgtggacgatggccgcgagcggccaccggctggctcgcttcgctcggcccgtggacaaccctgctggacaagctgatggacaggctgcgcctgcccacgagcttgaccacagggattgcccaccggctacccagccttcgaccacatacccaccggctccaactgcgcggcctgcggccttgccccatcaatttttttaattttctctggggaaaagcctccggcctgcggcctgcgcgcttcgcttgccggttggacaccaagtggaaggcgggtcaaggctcgcgcagcgaccgcgcagcggcttggccttgacgcgcctggaacgacccaagcctatgcgagtgggggcagtcgaaggcgaagcccgcccgcctgccccccgagcctcacggcggcgagtgcgggggttccaagggggcagcgccaccttgggcaaggccgaaggccgcgcagtcgatcaacaagccccggaggggccactttttgccggagggggagccgcgccgaaggcgtgggggaaccccgcaggggtgcccttctttgggcaccaaagaactagatatagggcgaaatgcgaaagacttaaaaatcaacaacttaaaaaaggggggtacgcaacagctcattgcggcaccccccgcaatagctcattgcgtaggttaaagaaaatctgtaattgactgccacttttacgcaacgcataattgttgtcgcgctgccgaaaagttgcagctgattgcgcatggtgccgcaaccgtgcggcaccctaccgcatggagataagcatggccacgcagtccagagaaatcggcattcaagccaagaacaagcccggtcactgggtgcaaacggaacgcaaagcgcatgaggcgtgggccgggcttattgcgaggaaacccacggcggcaatgctgctgcatcacctcgtggcgcagatgggccaccagaacgccgtggtggtcagccagaagacactttccaagctcatcggacgttctttgcggacggtccaatacgcagtcaaggacttggtggccgagcgctggatctccgtcgtgaagctcaacggccccggcaccgtgtcggcctacgtggtcaatgaccgcgtggcgtggggccagccccgcgaccagttgcgcctgtcggtgttcagtgccgccgtggtggttgatcacgacgaccaggacgaatcgctgttggggcatggcgacctgcgccgcatcccgaccctgtatccgggcgagcagcaactaccgaccggccccggcgaggagccgcccagccagcccggcattccgggcatggaaccagacctgccagccttgaccgaaacggaggaatgggaacggcgcgggcagcagcgcctgccgatgcccgatgagccgtgttttctggacgatggcgagccgttggagccgccgacacgggtcacgctgccgcgccggtagggcatcaaataaaacgaaaggctcagtcgaaagactgggcctttcgttttatctgttgtttgtcggtgaacgctctcctgagtaggacaaatccgccgccctagattaattaagcccattgacaaggctctcgcggccaggtataattgcacgacctagggtccaagttcacttaaaaaggagatcaacaatgaaagcaattttcgtactgaaacatcttaatcatgctaacgagattttctaatgtccaaaaccgttgaagagatctgggcagcccaacgcgctcgaggcccagctacagtgcttgcgatcggcaccgctgctcccgccaacgtggtgtaccaggcggactacccagactattatttccgcattaccaagagcgagcatatgaccgaattgaaggaaaagtttcgccggatgtgcgataagagtatgatcaccaagcgccatatgcatctgagtgaagagcttctgaaaaacaaccccgacatctgcgcgtacatggcgccctcgctcgacgcgcgtcaggacatggtggtggtggaagttccaaagctggggaaggaggctgccgcaaaagccatcaaagagtggggccggccgaagagcgccatcacccacctgattttctgcaccaccagcggcgtggacatgccgggcgccgacttccaactgactaagctgctcggcctatgcccgtcggtgcgccgcaccatgctgtaccagcaggggtgcttcgcgggcggtacagtgctgcgcctggccaaggatctggcggaaaacaatgcgggcgcccgcgtcctggtggtctgctcggaaatcaccgccgtgactttccgcggcccgtccgaaacccacctcgattcaatggttggccaggccttgtttggtgacggcgcctccgcgattatcgtgggcgccgacccggacccggtgattgagcgccctctcttccagatcgtctcggccgcccagaccattctgccggattcggacggtgcgatcgacgggcacctgcgggaggtgggcctgacctttcacctgctgaaggacgtaccgggcctgatcagcaagaacatcgagaagagcttgaaagaggccttcgccccgttaggcatcgacgattggaactcgatcttctggatcgtgcacccgggtggccctgcaatcctggatcaggtagaagccaagctccgtctgaagccggaaaagttgaaaaccaccaggacggtcctgtctgagtacgggaacatgagcagcgcctgtgtcttgttcatcctggatgagatgcgtcgtaacagcatggaagagggtaaagccacgactggcgaaggtctgcactggggcgtcctgttcgggttcggccccggactgacggtagagacggtcgtcctgcacagcttgcccatagcagaggcaaattgacttggactcctgttgatagatccagtaatgacctcagaactccatctggatttgttcagaacgctcggttgccgccgggcgttttttattggtgagaatccagattgcgttgcgctcactgcccgctttccagtcgggaaacctgtcgtgccagctgcattaatgaatcggccaacgcgcggggagaggcggtttgcgtattgggcgcatgcataaaaactgttgtaattcattaagcattctgccgacatggaagccatcacaaacggcatgatgaacctgaatcgccagcggcatcagcaccttgtcgccttgcgtataatatttgcccatgggggtgggcgaagaactccagcatgagatccccgcgctggaggatcatccagccggcgtcccggaaaacgattccgaagcccaacctttcatagaaggcggcggtggaatcgaaatctcgtgatggcaggttgggcgtcgcttggtcggtcatttcgaaccccagagtcccgctcagaagaactcgtcaagaaggcgatagaaggcgatgcgctgcgaatcgggagcggcgataccgtaaagcacgaggaagcggtcagcccattcgccgccaagctcttcagcaatatcacgggtagccaacgctatgtcctgatagcggtccgccacacccagccggccacagtcgatgaatccagaaaagcggccattttccaccatgatattcggcaagcaggcatcgccatgggtcacgacgagatcctcgccgtcgggcatgcgcgccttgagcctggcgaacagttcggctggcgcgagcccctgatgctcttcgtccagatcatcctgatcgacaagaccggcttccatccgagtacgtgctcgctcgatgcgatgtttcgcttggtggtcgaatgggcaggtagccggatcaagcgtatgcagccgccgcattgcatcagccatgatggatactttctcggcaggagcaaggtgagatgacaggagatcctgccccggcacttcgcccaatagcagccagtcccttcccgcttcagtgacaacgtcgagcacagctgcgcaaggaacgcccgtcgtggccagccacgatagccgcgctgcctcgtcctgcagttcattcagggcaccggacaggtcggtcttgacaaaaagaaccgggcgcccctgcgctgacagccggaacacggcggcatcagagcagccgattgtctgttgtgcccagtcatagccgaatagcctctccacccaagcggccggagaacctgcgtgcaatccatcttgttcaatcatgcgaaacgatcctcatcctgtctcttgatcagatcttgatcccctgcgccatcagatccttggcggcaagaaagccatccagtttactttgcagggcttcccaaccttaccagagggcgccccagctggcaattccggttcgcttgctgtccataaaaccgcccagtctagctatcgccatgtaagcccactgcaagctacctgctttctctttgcgcttgcgttttcccttgtccagatagcccagtagctgacattcatcccaggtggcacttttcggggaaatgtgcgcgcccgcgttcctgctggcgctgggcctgtttctggcgctggacttcccgctgttccgtcagcagcttttcgcccacggccttgatgatcgcggcggccttggcctgcatatcccgattcaacggccccagggcgtccagaacgggcttcaggcgctcccgaaggt

SEQ ID NO: 37 - DNA, 5642 bp, synthetic construct
  source 1..5642: mol_type = other DNA
ctcgggccgtctcttgggcttgatcggccttcttgcgcatctcacgcgctcctgcggcggcctgtagggcaggctcatacccctgccgaaccgcttttgtcagccggtcggccacggcttccggcgtctcaacgcgctttgagattcccagcttttcggccaatccctgcggtgcataggcgcgtggctcgaccgcttgcgggctgatggtgacgtggcccactggtggccgctccagggcctcgtagaacgcctgaatgcgcgtgtgacgtgccttgctgccctcgatgccccgttgcagccctagatcggccacagcggccgcaaacgtggtctggtcgcgggtcatctgcgctttgttgccgatgaactccttggccgacagcctgccgtcctgcgtcagcggcaccacgaacgcggtcatgtgcgggctggtttcgtcacggtggatgctggccgtcacgatgcgatccgccccgtacttgtccgccagccacttgtgcgccttctcgaagaacgccgcctgctgttcttggctggccgacttccaccattccgggctggccgtcatgacgtactcgaccgccaacacagcgtccttgcgccgcttctctggcagcaactcgcgcagtcggcccatcgcttcatcggtgctgctggccgcccagtgctcgttctctggcgtcctgctggcgtcagcgttgggcgtctcgcgctcgcggtaggcgtgcttgagactggccgccacgttgcccattttcgccagcttcttgcatcgcatgatcgcgtatgccgccatgcctgcccctcccttttggtgtccaaccggctcgacgggggcagcgcaaggcggtgcctccggcgggccactcaatgcttgagtatactcactagactttgcttcgcaaagtcgtgaccgcctacggcggctgcggcgccctacgggcttgctctccgggcttcgccctgcgcggtcgctgcgctcccttgccagcccgtggatatgtggacgatggccgcgagcggccaccggctggctcgcttcgctcggcccgtggacaaccctgctggacaagctgatggacaggctgcgcctgcccacgagcttgaccacagggattgcccaccggctacccagccttcgaccacatacccaccggctccaactgcgcggcctgcggccttgccccatcaatttttttaattttctctggggaaaagcctccggcctgcggcctgcgcgcttcgcttgccggttggacaccaagtggaaggcgggtcaaggctcgcgcagcgaccgcgcagcggcttggccttgacgcgcctggaacgacccaagcctatgcgagtgggggcagtcgaaggcgaagcccgcccgcctgccccccgagcctcacggcggcgagtgcgggggttccaagggggcagcgccaccttgggcaaggccgaaggccgcgcagtcgatcaacaagccccggaggggccactttttgccggagggggagccgcgccgaaggcgtgggggaaccccgcaggggtgcccttctttgggcaccaaagaactagatatagggcgaaatgcgaaagacttaaaaatcaacaacttaaaaaaggggggtacgcaacagctcattgcggcaccccccgcaatagctcattgcgtaggttaaagaaaatctgtaattgactgccacttttacgcaacgcataattgttgtcgcgctgccgaaaagttgcagctgattgcgcatggtgccgcaaccgtgcggcaccctaccgcatggagataagcatggccacgcagtccagagaaatcggcattcaagccaagaacaagcccggtcactgggtgcaaacggaacgcaaagcgcatgaggcgtgggccgggcttattgcgaggaaacccacggcggcaatgctgctgcatcacctcgtggcgcagatgggccaccagaacgccgtggtggtcagccagaagacactttccaagctcatcggacgttctttgcggacggtccaatacgcagtcaaggacttggtggccgagcgctggatctccgtcgtgaagctcaacggccccggcaccgtgtcggcctacgtggtcaatgaccgcgtggcgtggggccagccccgcgaccagttgcgcctgtcggtgttcagtgccgccgtggtggttgatcacgacgaccaggacgaatcgctgttggggcatggcgacctgcgccgcatcccgaccctgtatccgggcgagcagcaactaccgaccggccccggcgaggagccgcccagccagcccggcattccgggcatggaaccagacctgccagccttgaccgaaacggaggaatgggaacggcgcgggcagcagcgcctgccgatgcccgatgagccgtgttttctggacgatggcgagccgttggagccgccgacacgggtcacgctgccgcgccggtagggcatcaaataaaacgaaaggctcagtcgaaagactgggcctttcgttttatctgttgtttgtcggtgaacgctctcctgagtaggacaaatccgccgccctagattaattaagcccattgacaaggctctcgcggccaggtataattgcacgacctagggtccaagttcacttaaaaaggagatcaacaatgaaagcaattttcgtactgaaacatcttaatcatgctaacgagattttctaatgtccaaaaccgttgaagagatctgggcagcccaacgcgctcgaggcccagctacagtgcttgcgatcggcaccgctgctcccgccaacgtggtgtaccaggcggactacccagactattatttccgcattaccaagagcgagcatatgaccgaattgaaggaaaagtttcgccggatgtgcgataagagtcagatcaccaagcgccatatgcatctgagtgaagagcttctgaaaaacaaccccgacatctgcgcgtacatggcgccctcgctcgacgcgcgtcaggacatggtggtggtggaagttccaaagctggggaaggaggctgccgcaaaagccatcaaagagtggggccggccgaagagcgccatcacccacctgattttctgcaccaccagcggcgtggacatgccgggcgccgacttccaactgactaagctgctcggcctatgcccgtcggtgcgccgcaccatgctgtaccagcaggggtgcttcgcgggcggtacagtgctgcgcctggccaaggatctggcggaaaacaatgcgggcgcccgcgtcctggtggtctgctcggaaatcaccgccgtgactttccgcggcccgtccgaaacccacctcgattcaatggttggccaggccttgtttggtgacggcgcctccgcgattatcgtgggcgccgacccggacccggtgattgagcgccctctcttccagatcgtctcggccgcccagaccattctgccggattcggacggtgcgatcgacgggcacctgcgggaggtgggcctgacctttcacctgctgaaggacgtaccgggcctgatcagcaagaacatcgagaagagcttgaaagaggccttcgccccgttaggcatcgacgattggaactcgatcttctggatcgtgcacccgggtggccctgcaatcctggatcaggtagaagccaagctccgtctgaaggtcgaaaagttgaaaaccaccaggacggtcctgtctgagtacgggaacatgagcagcgcctgtgtcttgttcatcctggatgagatgcgtcgtaacagcatggaagagggtaaagccacgactggcgaaggtctgcactggggcgtcctgttcgggttcggccccggactgacggtagagacggtcgtcctgcacagcttgcccatagcagaggcaaattgacttggactcctgttgatagatccagtaatgacctcagaactccatctggatttgttcagaacgctcggttgccgccgggcgttttttattggtgagaatccagattgcgttgcgctcactgcccgctttccagtcgggaaacctgtcgtgccagctgcattaatgaatcggccaacgcgcggggagaggcggtttgcgtattgggcgcatgcataaaaactgttgtaattcattaagcattctgccgacatggaagccatcacaaacggcatgatgaacctgaatcgccagcggcatcagcaccttgtcgccttgcgtataatatttgcccatgggggtgggcgaagaactccagcatgagatccccgcgctggaggatcatccagccggcgtcccggaaaacgattccgaagcccaacctttcatagaaggcggcggtggaatcgaaatctcgtgatggcaggttgggcgtcgcttggtcggtcatttcgaaccccagagtcccgctcagaagaactcgtcaagaaggcgatagaaggcgatgcgctgcgaatcgggagcggcgataccgtaaagcacgaggaagcggtcagcccattcgccgccaagctcttcagcaatatcacgggtagccaacgctatgtcctgatagcggtccgccacacccagccggccacagtcgatgaatccagaaaagcggccattttccaccatgatattcggcaagcaggcatcgccatgggtcacgacgagatcctcgccgtcgggcatgcgcgccttgagcctggcgaacagttcggctggcgcgagcccctgatgctcttcgtccagatcatcctgatcgacaagaccggcttccatccgagtacgtgctcgctcgatgcgatgtttcgcttggtggtcgaatgggcaggtagccggatcaagcgtatgcagccgccgcattgcatcagccatgatggatactttctcggcaggagcaaggtgagatgacaggagatcctgccccggcacttcgcccaatagcagccagtcccttcccgcttcagtgacaacgtcgagcacagctgcgcaaggaacgcccgtcgtggccagccacgatagccgcgctgcctcgtcctgcagttcattcagggcaccggacaggtcggtcttgacaaaaagaaccgggcgcccctgcgctgacagccggaacacggcggcatcagagcagccgattgtctgttgtgcccagtcatagccgaatagcctctccacccaagcggccggagaacctgcgtgcaatccatcttgttcaatcatgcgaaacgatcctcatcctgtctcttgatcagatcttgatcccctgcgccatcagatccttggcggcaagaaagccatccagtttactttgcagggcttcccaaccttaccagagggcgccccagctggcaattccggttcgcttgctgtccataaaaccgcccagtctagctatcgccatgtaagcccactgcaagctacctgctttctctttgcgcttgcgttttcccttgtccagatagcccagtagctgacattcatcccaggtggcacttttcggggaaatgtgcgcgcccgcgttcctgctggcgctgggcctgtttctggcgctggacttcccgctgttccgtcagcagcttttcgcccacggccttgatgatcgcggcggccttggcctgcatatcccgattcaacggccccagggcgtccagaacgggcttcaggcgctcccgaaggt

SEQ ID NO: 38 - DNA, 5639 bp, synthetic construct
  source 1..5639: mol_type = other DNA
ctcgggccgtctcttgggcttgatcggccttcttgcgcatctcacgcgctcctgcggcggcctgtagggcaggctcatacccctgccgaaccgcttttgtcagccggtcggccacggcttccggcgtctcaacgcgctttgagattcccagcttttcggccaatccctgcggtgcataggcgcgtggctcgaccgcttgcgggctgatggtgacgtggcccactggtggccgctccagggcctcgtagaacgcctgaatgcgcgtgtgacgtgccttgctgccctcgatgccccgttgcagccctagatcggccacagcggccgcaaacgtggtctggtcgcgggtcatctgcgctttgttgccgatgaactccttggccgacagcctgccgtcctgcgtcagcggcaccacgaacgcggtcatgtgcgggctggtttcgtcacggtggatgctggccgtcacgatgcgatccgccccgtacttgtccgccagccacttgtgcgccttctcgaagaacgccgcctgctgttcttggctggccgacttccaccattccgggctggccgtcatgacgtactcgaccgccaacacagcgtccttgcgccgcttctctggcagcaactcgcgcagtcggcccatcgcttcatcggtgctgctggccgcccagtgctcgttctctggcgtcctgctggcgtcagcgttgggcgtctcgcgctcgcggtaggcgtgcttgagactggccgccacgttgcccattttcgccagcttcttgcatcgcatgatcgcgtatgccgccatgcctgcccctcccttttggtgtccaaccggctcgacgggggcagcgcaaggcggtgcctccggcgggccactcaatgcttgagtatactcactagactttgcttcgcaaagtcgtgaccgcctacggcggctgcggcgccctacgggcttgctctccgggcttcgccctgcgcggtcgctgcgctcccttgccagcccgtggatatgtggacgatggccgcgagcggccaccggctggctcgcttcgctcggcccgtggacaaccctgctggacaagctgatggacaggctgcgcctgcccacgagcttgaccacagggattgcccaccggctacccagccttcgaccacatacccaccggctccaactgcgcggcctgcggccttgccccatcaatttttttaattttctctggggaaaagcctccggcctgcggcctgcgcgcttcgcttgccggttggacaccaagtggaaggcgggtcaaggctcgcgcagcgaccgcgcagcggcttggccttgacgcgcctggaacgacccaagcctatgcgagtgggggcagtcgaaggcgaagcccgcccgcctgccccccgagcctcacggcggcgagtgcgggggttccaagggggcagcgccaccttgggcaaggccgaaggccgcgcagtcgatcaacaagccccggaggggccactttttgccggagggggagccgcgccgaaggcgtgggggaaccccgcaggggtgcccttctttgggcaccaaagaactagatatagggcgaaatgcgaaagacttaaaaatcaacaacttaaaaaaggggggtacgcaacagctcattgcggcaccccccgcaatagctcattgcgtaggttaaagaaaatctgtaattgactgccacttttacgcaacgcataattgttgtcgcgctgccgaaaagttgcagctgattgcgcatggtgccgcaaccgtgcggcaccctaccgcatggagataagcatggccacgcagtccagagaaatcggcattcaagccaagaacaagcccggtcactgggtgcaaacggaacgcaaagcgcatgaggcgtgggccgggcttattgcgaggaaacccacggcggcaatgctgctgcatcacctcgtggcgcagatgggccaccagaacgccgtggtggtcagccagaagacactttccaagctcatcggacgttctttgcggacggtccaatacgcagtcaaggacttggtggccgagcgctggatctccgtcgtgaagctcaacggccccggcaccgtgtcggcctacgtggtcaatgaccgcgtggcgtggggccagccccgcgaccagttgcgcctgtcggtgttcagtgccgccgtggtggttgatcacgacgaccaggacgaatcgctgttggggcatggcgacctgcgccgcatcccgaccctgtatccgggcgagcagcaactaccgaccggccccggcgaggagccgcccagccagcccggcattccgggcatggaaccagacctgccagccttgaccgaaacggaggaatgggaacggcgcgggcagcagcgcctgccgatgcccgatgagccgtgttttctggacgatggcgagccgttggagccgccgacacgggtcacgctgccgcgccggtagggcatcaaataaaacgaaaggctcagtcgaaagactgggcctttcgttttatctgttgtttgtcggtgaacgctctcctgagtaggacaaatccgccgccctagattaattaagcccattgacaaggctctcgcggccaggtataattgcacgacctagggcccaagttcacttaaaaaggagatcaacaatgaaagcaattttcgtactgaaacatcttaatcatgctaacgagattttctaatggtttctgtgggcgaaatccgcaagagccagcgtgcagagggcccggcaactgtactcgccatcggcaccgccacgcccgccaactgcgtgtaccaggcggactacccggactactacttccgaatcaccaacagtgaacacatgactgagctaaaagagaagttcaaacgtatgtgcgataagagcatgatcaacaagcgctacatgcacctgaacgaggagatccttaaggagaaccccaacgtttgcgcgtacatggccccgtcgctggacgctcgccaggatatggtggtggtggaggtgccaaaattgggcaaggaagcggccgtaaaggctattaaggagtggggtcagcctaagagcaagatcacgcatctggttttctgcacgaccagcggcgtggatatgcctggtgccgactatcagttgacgaagcttctgggtttgaagccgagcgtaaaacgcctcatgatgtatcagcagggctgtttcgccggcgggaccgtgttgcgcttggctaaagacctcgctgagaataacgccggcgcccgcgtgctcgtggtctgctcagagattaccgccgtcaccttccgtgggccctcggatacccacctggatagcttggtgggtcaggccctgttcggtgacggcgccgcggccattattatcggcgcggacccggacacaaagatcgaacgccccctgttcgaactggtctccgcggcccaaaccatccttccggatagcgaaggtgccatcgacggccacctgcgggaagtcggtctgaccttccacctgctgaaagacgtcccgggcctgatctcgaaaaacatcgagaaatcgctggtcgaggcgttcaagccgatcggcatctccgactggaattcgctgttctggatcgcgcatccaggcggcccggccatcctggaccaagtggagctcaagctgggcctgaaggaggagaagctgcgggccaccaggcatgtgctgtccgaatatgggaacatgagctccgcatgcgtcctgtttattctggacgaaatgcgcaagaagtcgatagaagaaggcaaggggaccacaggcgaagggctggaatggggcgtgctgtttggctttggcccaggactgaccgtcgaaaccgtcgtgctgcacagcctggcaacccaaagtacccactgacttggactcctgttgatagatccagtaatgacctcagaactccatctggatttgttcagaacgctcggttgccgccgggcgttttttattggtgagaatccagattgcgttgcgctcactgcccgctttccagtcgggaaacctgtcgtgccagctgcattaatgaatcggccaacgcgcggggagaggcggtttgcgtattgggcgcatgcataaaaactgttgtaattcattaagcattctgccgacatggaagccatcacaaacggcatgatgaacctgaatcgccagcggcatcagcaccttgtcgccttgcgtataatatttgcccatgggggtgggcgaagaactccagcatgagatccccgcgctggaggatcatccagccggcgtcccggaaaacgattccgaagcccaacctttcatagaaggcggcggtggaatcgaaatctcgtgatggcaggttgggcgtcgcttggtcggtcatttcgaaccccagagtcccgctcagaagaactcgtcaagaaggcgatagaaggcgatgcgctgcgaatcgggagcggcgataccgtaaagcacgaggaagcggtcagcccattcgccgccaagctcttcagcaatatcacgggtagccaacgctatgtcctgatagcggtccgccacacccagccggccacagtcgatgaatccagaaaagcggccattttccaccatgatattcggcaagcaggcatcgccatgggtcacgacgagatcctcgccgtcgggcatgcgcgccttgagcctggcgaacagttcggctggcgcgagcccctgatgctcttcgtccagatcatcctgatcgacaagaccggcttccatccgagtacgtgctcgctcgatgcgatgtttcgcttggtggtcgaatgggcaggtagccggatcaagcgtatgcagccgccgcattgcatcagccatgatggatactttctcggcaggagcaaggtgagatgacaggagatcctgccccggcacttcgcccaatagcagccagtcccttcccgcttcagtgacaacgtcgagcacagctgcgcaaggaacgcccgtcgtggccagccacgatagccgcgctgcctcgtcctgcagttcattcagggcaccggacaggtcggtcttgacaaaaagaaccgggcgcccctgcgctgacagccggaacacggcggcatcagagcagccgattgtctgttgtgcccagtcatagccgaatagcctctccacccaagcggccggagaacctgcgtgcaatccatcttgttcaatcatgcgaaacgatcctcatcctgtctcttgatcagatcttgatcccctgcgccatcagatccttggcggcaagaaagccatccagtttactttgcagggcttcccaaccttaccagagggcgccccagctggcaattccggttcgcttgctgtccataaaaccgcccagtctagctatcgccatgtaagcccactgcaagctacctgctttctctttgcgcttgcgttttcccttgtccagatagcccagtagctgacattcatcccaggtggcacttttcggggaaatgtgcgcgcccgcgttcctgctggcgctgggcctgtttctggcgctggacttcccgctgttccgtcagcagcttttcgcccacggccttgatgatcgcggcggccttggcctgcatatcccgattcaacggccccagggcgtccagaacgggcttcaggcgctcccgaaggt

SEQ ID NO: 39 - DNA, 5639 bp, synthetic construct
  source 1..5639: mol_type = other DNA
ctcgggccgtctcttgggcttgatcggccttcttgcgcatctcacgcgctcctgcggcggcctgtagggcaggctcatacccctgccgaaccgcttttgtcagccggtcggccacggcttccggcgtctcaacgcgctttgagattcccagcttttcggccaatccctgcggtgcataggcgcgtggctcgaccgcttgcgggctgatggtgacgtggcccactggtggccgctccagggcctcgtagaacgcctgaatgcgcgtgtgacgtgccttgctgccctcgatgccccgttgcagccctagatcggccacagcggccgcaaacgtggtctggtcgcgggtcatctgcgctttgttgccgatgaactccttggccgacagcctgccgtcctgcgtcagcggcaccacgaacgcggtcatgtgcgggctggtttcgtcacggtggatgctggccgtcacgatgcgatccgccccgtacttgtccgccagccacttgtgcgccttctcgaagaacgccgcctgctgttcttggctggccgacttccaccattccgggctggccgtcatgacgtactcgaccgccaacacagcgtccttgcgccgcttctctggcagcaactcgcgcagtcggcccatcgcttcatcggtgctgctggccgcccagtgctcgttctctggcgtcctgctggcgtcagcgttgggcgtctcgcgctcgcggtaggcgtgcttgagactggccgccacgttgcccattttcgccagcttcttgcatcgcatgatcgcgtatgccgccatgcctgcccctcccttttggtgtccaaccggctcgacgggggcagcgcaaggcggtgcctccggcgggccactcaatgcttgagtatactcactagactttgcttcgcaaagtcgtgaccgcctacggcggctgcggcgccctacgggcttgctctccgggcttcgccctgcgcggtcgctgcgctcccttgccagcccgtggatatgtggacgatggccgcgagcggccaccggctggctcgcttcgctcggcccgtggacaaccctgctggacaagctgatggacaggctgcgcctgcccacgagcttgaccacagggattgcccaccggctacccagccttcgaccacatacccaccggctccaactgcgcggcctgcggccttgccccatcaatttttttaattttctctggggaaaagcctccggcctgcggcctgcgcgcttcgcttgccggttggacaccaagtggaaggcgggtcaaggctcgcgcagcgaccgcgcagcggcttggccttgacgcgcctggaacgacccaagcctatgcgagtgggggcagtcgaaggcgaagcccgcccgcctgccccccgagcctcacggcggcgagtgcgggggttccaagggggcagcgccaccttgggcaaggccgaaggccgcgcagtcgatcaacaagccccggaggggccactttttgccggagggggagccgcgccgaaggcgtgggggaaccccgcaggggtgcccttctttgggcaccaaagaactagatatagggcgaaatgcgaaagacttaaaaatcaacaacttaaaaaaggggggtacgcaacagctcattgcggcaccccccgcaatagctcattgcgtaggttaaagaaaatctgtaattgactgccacttttacgcaacgcataattgttgtcgcgctgccgaaaagttgcagctgattgcgcatggtgccgcaaccgtgcggcaccctaccgcatggagataagcatggccacgcagtccagagaaatcggcattcaagccaagaacaagcccggtcactgggtgcaaacggaacgcaaagcgcatgaggcgtgggccgggcttattgcgaggaaacccacggcggcaatgctgctgcatcacctcgtggcgcagatgggccaccagaacgccgtggtggtcagccagaagacactttccaagctcatcggacgttctttgcggacggtccaatacgcagtcaaggacttggtggccgagcgctggatctccgtcgtgaagctcaacggccccggcaccgtgtcggcctacgtggtcaatgaccgcgtggcgtggggccagccccgcgaccagttgcgcctgtcggtgttcagtgccgccgtggtggttgatcacgacgaccaggacgaatcgctgttggggcatggcgacctgcgccgcatcccgaccctgtatccgggcgagcagcaactaccgaccggccccggcgaggagccgcccagccagcccggcattccgggcatggaaccagacctgccagccttgaccgaaacggaggaatgggaacggcgcgggcagcagcgcctgccgatgcccgatgagccgtgttttctggacgatggcgagccgttggagccgccgacacgggtcacgctgccgcgccggtagggcatcaaataaaacgaaaggctcagtcgaaagactgggcctttcgttttatctgttgtttgtcggtgaacgctctcctgagtaggacaaatccgccgccctagattaattaagcccattgacaaggctctcgcggccaggtataattgcacgacctagggcccaagttcacttaaaaaggagatcaacaatgaaagcaattttcgtactgaaacatcttaatcatgctaacgagattttctaatggtttctgtgggcgaaatccgcaagagccagcgtgcagagggcccggcaactgtactcgccatcggcaccgccacgcccgccaactgcgtgtaccaggcggactacccggactactacttccgaatcaccaacagtgaacacatgactgagctaaaagagaagttcaaacgtatgtgcgataagagcatgatcaacaagcgctacatgcacctgaacgaggagatccttaaggagaaccccaacgtttgcgcgtacatggccccgtcgctggacgctcgccaggatatggtggtggtggaggtgccaaaattgggcaaggaagcggccgtaaaggctattaaggagtggggtcagcctaagagcaagatcacgcatctggttttctgcacgaccagcggcgtggatatgcctggtgccgactatcagttgacgaagcttctgggtttgaagccgagcgtaaaacgcctcatgatgtatcagcagggctgtttcgccggcgggaccgtgttgcgcttggctaaagacctcgctgagaataacgccggcgcccgcgtgctcgtggtctgctcagagattaccgccgtcaccttccgtgggccctcggatacccacctggatagcttggtgggtcaggccctgttcggtgacggcgccgcggccattattatcggcgcggacccggacacaaagatcgaacgccccctgttcgaactggtctccgcggcccaaaccatccttccggatagcgaaggtgccatcgacggccacctgcgggaagtcggtctgaccttccacctgctgaaagacgtcccgggcctgatctcgaaaaacatcgagaaatcgctggtcgaggcgttcgccccgatcggcatctccgactggaattcgctgttctggatcgcgcatccaggcggcccggccatcctggaccaagtggagctcaagctgggcctgaaggaggagaagctgcgggccaccaggcatgtgctgtccgaatatgggaacatgagctccgcatgcgtcctgtttattctggacgaaatgcgcaagaagtcgatagaagaaggcaaggggaccacaggcgaagggctggaatggggcgtgctgtttggctttggcccaggactgaccgtcgaaaccgtcgtgctgcacagcctggcaacccaaagtacccactgacttggactcctgttgatagatccagtaatgacctcagaactccatctggatttgttcagaacgctcggttgccgccgggcgttttttattggtgagaatccagattgcgttgcgctcactgcccgctttccagtcgggaaacctgtcgtgccagctgcattaatgaatcggccaacgcgcggggagaggcggtttgcgtattgggcgcatgcataaaaactgttgtaattcattaagcattctgccgacatggaagccatcacaaacggcatgatgaacctgaatcgccagcggcatcagcaccttgtcgccttgcgtataatatttgcccatgggggtgggcgaagaactccagcatgagatccccgcgctggaggatcatccagccggcgtcccggaaaacgattccgaagcccaacctttcatagaaggcggcggtggaatcgaaatctcgtgatggcaggttgggcgtcgcttggtcggtcatttcgaaccccagagtcccgctcagaagaactcgtcaagaaggcgatagaaggcgatgcgctgcgaatcgggagcggcgataccgtaaagcacgaggaagcggtcagcccattcgccgccaagctcttcagcaatatcacgggtagccaacgctatgtcctgatagcggtccgccacacccagccggccacagtcgatgaatccagaaaagcggccattttccaccatgatattcggcaagcaggcatcgccatgggtcacgacgagatcctcgccgtcgggcatgcgcgccttgagcctggcgaacagttcggctggcgcgagcccctgatgctcttcgtccagatcatcctgatcgacaagaccggcttccatccgagtacgtgctcgctcgatgcgatgtttcgcttggtggtcgaatgggcaggtagccggatcaagcgtatgcagccgccgcattgcatcagccatgatggatactttctcggcaggagcaaggtgagatgacaggagatcctgccccggcacttcgcccaatagcagccagtcccttcccgcttcagtgacaacgtcgagcacagctgcgcaaggaacgcccgtcgtggccagccacgatagccgcgctgcctcgtcctgcagttcattcagggcaccggacaggtcggtcttgacaaaaagaaccgggcgcccctgcgctgacagccggaacacggcggcatcagagcagccgattgtctgttgtgcccagtcatagccgaatagcctctccacccaagcggccggagaacctgcgtgcaatccatcttgttcaatcatgcgaaacgatcctcatcctgtctcttgatcagatcttgatcccctgcgccatcagatccttggcggcaagaaagccatccagtttactttgcagggcttcccaaccttaccagagggcgccccagctggcaattccggttcgcttgctgtccataaaaccgcccagtctagctatcgccatgtaagcccactgcaagctacctgctttctctttgcgcttgcgttttcccttgtccagatagcccagtagctgacattcatcccaggtggcacttttcggggaaatgtgcgcgcccgcgttcctgctggcgctgggcctgtttctggcgctggacttcccgctgttccgtcagcagcttttcgcccacggccttgatgatcgcggcggccttggcctgcatatcccgattcaacggccccagggcgtccagaacgggcttcaggcgctcccgaaggt

SEQ ID NO: 40 - DNA, 5639 bp, synthetic construct
  source 1..5639: mol_type = other DNA
ctcgggccgtctcttgggcttgatcggccttcttgcgcatctcacgcgctcctgcggcggcctgtagggcaggctcatacccctgccgaaccgcttttgtcagccggtcggccacggcttccggcgtctcaacgcgctttgagattcccagcttttcggccaatccctgcggtgcataggcgcgtggctcgaccgcttgcgggctgatggtgacgtggcccactggtggccgctccagggcctcgtagaacgcctgaatgcgcgtgtgacgtgccttgctgccctcgatgccccgttgcagccctagatcggccacagcggccgcaaacgtggtctggtcgcgggtcatctgcgctttgttgccgatgaactccttggccgacagcctgccgtcctgcgtcagcggcaccacgaacgcggtcatgtgcgggctggtttcgtcacggtggatgctggccgtcacgatgcgatccgccccgtacttgtccgccagccacttgtgcgccttctcgaagaacgccgcctgctgttcttggctggccgacttccaccattccgggctggccgtcatgacgtactcgaccgccaacacagcgtccttgcgccgcttctctggcagcaactcgcgcagtcggcccatcgcttcatcggtgctgctggccgcccagtgctcgttctctggcgtcctgctggcgtcagcgttgggcgtctcgcgctcgcggtaggcgtgcttgagactggccgccacgttgcccattttcgccagcttcttgcatcgcatgatcgcgtatgccgccatgcctgcccctcccttttggtgtccaaccggctcgacgggggcagcgcaaggcggtgcctccggcgggccactcaatgcttgagtatactcactagactttgcttcgcaaagtcgtgaccgcctacggcggctgcggcgccctacgggcttgctctccgggcttcgccctgcgcggtcgctgcgctcccttgccagcccgtggatatgtggacgatggccgcgagcggccaccggctggctcgcttcgctcggcccgtggacaaccctgctggacaagctgatggacaggctgcgcctgcccacgagcttgaccacagggattgcccaccggctacccagccttcgaccacatacccaccggctccaactgcgcggcctgcggccttgccccatcaatttttttaattttctctggggaaaagcctccggcctgcggcctgcgcgcttcgcttgccggttggacaccaagtggaaggcgggtcaaggctcgcgcagcgaccgcgcagcggcttggccttgacgcgcctggaacgacccaagcctatgcgagtgggggcagtcgaaggcgaagcccgcccgcctgccccccgagcctcacggcggcgagtgcgggggttccaagggggcagcgccaccttgggcaaggccgaaggccgcgcagtcgatcaacaagccccggaggggccactttttgccggagggggagccgcgccgaaggcgtgggggaaccccgcaggggtgcccttctttgggcaccaaagaactagatatagggcgaaatgcgaaagacttaaaaatcaacaacttaaaaaaggggggtacgcaacagctcattgcggcaccccccgcaatagctcattgcgtaggttaaagaaaatctgtaattgactgccacttttacgcaacgcataattgttgtcgcgctgccgaaaagttgcagctgattgcgcatggtgccgcaaccgtgcggcaccctaccgcatggagataagcatggccacgcagtccagagaaatcggcattcaagccaagaacaagcccggtcactgggtgcaaacggaacgcaaagcgcatgaggcgtgggccgggcttattgcgaggaaacccacggcggcaatgctgctgcatcacctcgtggcgcagatgggccaccagaacgccgtggtggtcagccagaagacactttccaagctcatcggacgttctttgcggacggtccaatacgcagtcaaggacttggtggccgagcgctggatctccgtcgtgaagctcaacggccccggcaccgtgtcggcctacgtggtcaatgaccgcgtggcgtggggccagccccgcgaccagttgcgcctgtcggtgttcagtgccgccgtggtggttgatcacgacgaccaggacgaatcgctgttggggcatggcgacctgcgccgcatcccgaccctgtatccgggcgagcagcaactaccgaccggccccggcgaggagccgcccagccagcccggcattccgggcatggaaccagacctgccagccttgaccgaaacggaggaatgggaacggcgcgggcagcagcgcctgccgatgcccgatgagccgtgttttctggacgatggcgagccgttggagccgccgacacgggtcacgctgccgcgccggtagggcatcaaataaaacgaaaggctcagtcgaaagactgggcctttcgttttatctgttgtttgtcggtgaacgctctcctgagtaggacaaatccgccgccctagattaattaagcccattgacaaggctctcgcggccaggtataattgcacgacctagggcccaagttcacttaaaaaggagatcaacaatgaaagcaattttcgtactgaaacatcttaatcatgctaacgagattttctaatggtttctgtgggcgaaatccgcaagagccagcgtgcagagggcccggcaactgtactcgccatcggcaccgccacgcccgccaactgcgtgtaccaggcggactacgccgactactacttccgaatcaccaacagtgaacacatgactgagctaaaagagaagttcaaacgtatgtgcgataagagcatgatcaacaagcgctacatgcacctgaacgaggagatccttaaggagaaccccaacgtttgcgcgtacatggccccgtcgctggacgctcgccaggatatggtggtggtggaggtgccaaaattgggcaaggaagcggccgtaaaggctattaaggagtggggtcagcctaagagcaagatcacgcatctggttttctgcacgaccagcggcgtggatatgcctggtgccgactatcagttgacgaagcttctgggtttgaagccgagcgtaaaacgcctcatgatgtatcagcagggctgtttcgccggcgggaccgtgttgcgcttggctaaagacctcgctgagaataacgccggcgcccgcgtgctcgtggtctgctcagagattaccgccgtcaccttccgtgggccctcggatacccacctggatagcttggtgggtcaggccctgttcggtgacggcgccgcggccattattatcggcgcggacccggacacaaagatcgaacgccccctgttcgaactggtctccgcggcccaaaccatccttccggatagcgaaggtgccatcgacggccacctgcgggaagtcggtctgaccttccacctgctgaaagacgtcccgggcctgatctcgaaaaacatcgagaaatcgctggtcgaggcgttcaagccgatcggcatctccgactggaattcgctgttctggatcgcgcatccaggcggcccggccatcctggaccaagtggagctcaagctgggcctgaaggaggagaagctgcgggccaccaggcatgtgctgtccgaatatgggaacatgagctccgcatgcgtcctgtttattctggacgaaatgcgcaagaagtcgatagaagaaggcaaggggaccacaggcgaagggctggaatggggcgtgctgtttggctttggcccaggactgaccgtcgaaaccgtcgtgctgcacagcctggcaacccaaagtacccactgacttggactcctgttgatagatccagtaatgacctcagaactccatctggatttgttcagaacgctcggttgccgccgggcgttttttattggtgagaatccagattgcgttgcgctcactgcccgctttccagtcgggaaacctgtcgtgccagctgcattaatgaatcggccaacgcgcggggagaggcggtttgcgtattgggcgcatgcataaaaactgttgtaattcattaagcattctgccgacatggaagccatcacaaacggcatgatgaacctgaatcgccagcggcatcagcaccttgtcgccttgcgtataatatttgcccatgggggtgggcgaagaactccagcatgagatccccgcgctggaggatcatccagccggcgtcccggaaaacgattccgaagcccaacctttcatagaaggcggcggtggaatcgaaatctcgtgatggcaggttgggcgtcgcttggtcggtcatttcgaaccccagagtcccgctcagaagaactcgtcaagaaggcgatagaaggcgatgcgctgcgaatcgggagcggcgataccgtaaagcacgaggaagcggtcagcccattcgccgccaagctcttcagcaatatcacgggtagccaacgctatgtcctgatagcggtccgccacacccagccggccacagtcgatgaatccagaaaagcggccattttccaccatgatattcggcaagcaggcatcgccatgggtcacgacgagatcctcgccgtcgggcatgcgcgccttgagcctggcgaacagttcggctggcgcgagcccctgatgctcttcgtccagatcatcctgatcgacaagaccggcttccatccgagtacgtgctcgctcgatgcgatgtttcgcttggtggtcgaatgggcaggtagccggatcaagcgtatgcagccgccgcattgcatcagccatgatggatactttctcggcaggagcaaggtgagatgacaggagatcctgccccggcacttcgcccaatagcagccagtcccttcccgcttcagtgacaacgtcgagcacagctgcgcaaggaacgcccgtcgtggccagccacgatagccgcgctgcctcgtcctgcagttcattcagggcaccggacaggtcggtcttgacaaaaagaaccgggcgcccctgcgctgacagccggaacacggcggcatcagagcagccgattgtctgttgtgcccagtcatagccgaatagcctctccacccaagcggccggagaacctgcgtgcaatccatcttgttcaatcatgcgaaacgatcctcatcctgtctcttgatcagatcttgatcccctgcgccatcagatccttggcggcaagaaagccatccagtttactttgcagggcttcccaaccttaccagagggcgccccagctggcaattccggttcgcttgctgtccataaaaccgcccagtctagctatcgccatgtaagcccactgcaagctacctgctttctctttgcgcttgcgttttcccttgtccagatagcccagtagctgacattcatcccaggtggcacttttcggggaaatgtgcgcgcccgcgttcctgctggcgctgggcctgtttctggcgctggacttcccgctgttccgtcagcagcttttcgcccacggccttgatgatcgcggcggccttggcctgcatatcccgattcaacggccccagggcgtccagaacgggcttcaggcgctcccgaaggt

SEQ ID NO: 41 - DNA, 5639 bp, synthetic construct
  source 1..5639: mol_type = other DNA
ctcgggccgtctcttgggcttgatcggccttcttgcgcatctcacgcgctcctgcggcggcctgtagggcaggctcatacccctgccgaaccgcttttgtcagccggtcggccacggcttccggcgtctcaacgcgctttgagattcccagcttttcggccaatccctgcggtgcataggcgcgtggctcgaccgcttgcgggctgatggtgacgtggcccactggtggccgctccagggcctcgtagaacgcctgaatgcgcgtgtgacgtgccttgctgccctcgatgccccgttgcagccctagatcggccacagcggccgcaaacgtggtctggtcgcgggtcatctgcgctttgttgccgatgaactccttggccgacagcctgccgtcctgcgtcagcggcaccacgaacgcggtcatgtgcgggctggtttcgtcacggtggatgctggccgtcacgatgcgatccgccccgtacttgtccgccagccacttgtgcgccttctcgaagaacgccgcctgctgttcttggctggccgacttccaccattccgggctggccgtcatgacgtactcgaccgccaacacagcgtccttgcgccgcttctctggcagcaactcgcgcagtcggcccatcgcttcatcggtgctgctggccgcccagtgctcgttctctggcgtcctgctggcgtcagcgttgggcgtctcgcgctcgcggtaggcgtgcttgagactggccgccacgttgcccattttcgccagcttcttgcatcgcatgatcgcgtatgccgccatgcctgcccctcccttttggtgtccaaccggctcgacgggggcagcgcaaggcggtgcctccggcgggccactcaatgcttgagtatactcactagactttgcttcgcaaagtcgtgaccgcctacggcggctgcggcgccctacgggcttgctctccgggcttcgccctgcgcggtcgctgcgctcccttgccagcccgtggatatgtggacgatggccgcgagcggccaccggctggctcgcttcgctcggcccgtggacaaccctgctggacaagctgatggacaggctgcgcctgcccacgagcttgaccacagggattgcccaccggctacccagccttcgaccacatacccaccggctccaactgcgcggcctgcggccttgccccatcaatttttttaattttctctggggaaaagcctccggcctgcggcctgcgcgcttcgcttgccggttggacaccaagtggaaggcgggtcaaggctcgcgcagcgaccgcgcagcggcttggccttgacgcgcctggaacgacccaagcctatgcgagtgggggcagtcgaaggcgaagcccgcccgcctgccccccgagcctcacggcggcgagtgcgggggttccaagggggcagcgccaccttgggcaaggccgaaggccgcgcagtcgatcaacaagccccggaggggccactttttgccggagggggagccgcgccgaaggcgtgggggaaccccgcaggggtgcccttctttgggcaccaaagaactagatatagggcgaaatgcgaaagacttaaaaatcaacaacttaaaaaaggggggtacgcaacagctcattgcggcaccccccgcaatagctcattgcgtaggttaaagaaaatctgtaattgactgccacttttacgcaacgcataattgttgtcgcgctgccgaaaagttgcagctgattgcgcatggtgccgcaaccgtgcggcaccctaccgcatggagataagcatggccacgcagtccagagaaatcggcattcaagccaagaacaagcccggtcactgggtgcaaacggaacgcaaagcgcatgaggcgtgggccgggcttattgcgaggaaacccacggcggcaatgctgctgcatcacctcgtggcgcagatgggccaccagaacgccgtggtggtcagccagaagacactttccaagctcatcggacgttctttgcggacggtccaatacgcagtcaaggacttggtggccgagcgctggatctccgtcgtgaagctcaacggccccggcaccgtgtcggcctacgtggtcaatgaccgcgtggcgtggggccagccccgcgaccagttgcgcctgtcggtgttcagtgccgccgtggtggttgatcacgacgaccaggacgaatcgctgttggggcatggcgacctgcgccgcatcccgaccctgtatccgggcgagcagcaactaccgaccggccccggcgaggagccgcccagccagcccggcattccgggcatggaaccagacctgccagccttgaccgaaacggaggaatgggaacggcgcgggcagcagcgcctgccgatgcccgatgagccgtgttttctggacgatggcgagccgttggagccgccgacacgggtcacgctgccgcgccggtagggcatcaaataaaacgaaaggctcagtcgaaagactgggcctttcgttttatctgttgtttgtcggtgaacgctctcctgagtaggacaaatccgccgccctagattaattaagcccattgacaaggctctcgcggccaggtataattgcacgacctagggcccaagttcacttaaaaaggagatcaacaatgaaagcaattttcgtactgaaacatcttaatcatgctaacgagattttctaatggtttctgtgggcgaaatccgcaagagccagcgtgcagagggcccggcaactgtactcgccatcggcaccgccacgcccgccaactgcgtgtaccaggcggactacccggactactacttccgaatcaccaacagtgaacacatgactgagctaaaagagaagttcaaacgtatgtgcgataagagccagatcaacaagcgctacatgcacctgaacgaggagatccttaaggagaaccccaacgtttgcgcgtacatggccccgtcgctggacgctcgccaggatatggtggtggtggaggtgccaaaattgggcaaggaagcggccgtaaaggctattaaggagtggggtcagcctaagagcaagatcacgcatctggttttctgcacgaccagcggcgtggatatgcctggtgccgactatcagttgacgaagcttctgggtttgaagccgagcgtaaaacgcctcatgatgtatcagcagggctgtttcgccggcgggaccgtgttgcgcttggctaaagacctcgctgagaataacgccggcgcccgcgtgctcgtggtctgctcagagattaccgccgtcaccttccgtgggccctcggatacccacctggatagcttggtgggtcaggccctgttcggtgacggcgccgcggccattattatcggcgcggacccggacacaaagatcgaacgccccctgttcgaactggtctccgcggcccaaaccatccttccggatagcgaaggtgccatcgacggccacctgcgggaagtcggtctgaccttccacctgctgaaagacgtcccgggcctgatctcgaaaaacatcgagaaatcgctggtcgaggcgttcaagccgatcggcatctccgactggaattcgctgttctggatcgcgcatccaggcggcccggccatcctggaccaagtggagctcaagctgggcctgaaggaggagaagctgcgggccaccaggcatgtgctgtccgaatatgggaacatgagctccgcatgcgtcctgtttattctggacgaaatgcgcaagaagtcgatagaagaaggcaaggggaccacaggcgaagggctggaatggggcgtgctgtttggctttggcccaggactgaccgtcgaaaccgtcgtgctgcacagcctggcaacccaaagtacccactgacttggactcctgttgatagatccagtaatgacctcagaactccatctggatttgttcagaacgctcggttgccgccgggcgttttttattggtgagaatccagattgcgttgcgctcactgcccgctttccagtcgggaaacctgtcgtgccagctgcattaatgaatcggccaacgcgcggggagaggcggtttgcgtattgggcgcatgcataaaaactgttgtaattcattaagcattctgccgacatggaagccatcacaaacggcatgatgaacctgaatcgccagcggcatcagcaccttgtcgccttgcgtataatatttgcccatgggggtgggcgaagaactccagcatgagatccccgcgctggaggatcatccagccggcgtcccggaaaacgattccgaagcccaacctttcatagaaggcggcggtggaatcgaaatctcgtgatggcaggttgggcgtcgcttggtcggtcatttcgaaccccagagtcccgctcagaagaactcgtcaagaaggcgatagaaggcgatgcgctgcgaatcgggagcggcgataccgtaaagcacgaggaagcggtcagcccattcgccgccaagctcttcagcaatatcacgggtagccaacgctatgtcctgatagcggtccgccacacccagccggccacagtcgatgaatccagaaaagcggccattttccaccatgatattcggcaagcaggcatcgccatgggtcacgacgagatcctcgccgtcgggcatgcgcgccttgagcctggcgaacagttcggctggcgcgagcccctgatgctcttcgtccagatcatcctgatcgacaagaccggcttccatccgagtacgtgctcgctcgatgcgatgtttcgcttggtggtcgaatgggcaggtagccggatcaagcgtatgcagccgccgcattgcatcagccatgatggatactttctcggcaggagcaaggtgagatgacaggagatcctgccccggcacttcgcccaatagcagccagtcccttcccgcttcagtgacaacgtcgagcacagctgcgcaaggaacgcccgtcgtggccagccacgatagccgcgctgcctcgtcctgcagttcattcagggcaccggacaggtcggtcttgacaaaaagaaccgggcgcccctgcgctgacagccggaacacggcggcatcagagcagccgattgtctgttgtgcccagtcatagccgaatagcctctccacccaagcggccggagaacctgcgtgcaatccatcttgttcaatcatgcgaaacgatcctcatcctgtctcttgatcagatcttgatcccctgcgccatcagatccttggcggcaagaaagccatccagtttactttgcagggcttcccaaccttaccagagggcgccccagctggcaattccggttcgcttgctgtccataaaaccgcccagtctagctatcgccatgtaagcccactgcaagctacctgctttctctttgcgcttgcgttttcccttgtccagatagcccagtagctgacattcatcccaggtggcacttttcggggaaatgtgcgcgcccgcgttcctgctggcgctgggcctgtttctggcgctggacttcccgctgttccgtcagcagcttttcgcccacggccttgatgatcgcggcggccttggcctgcatatcccgattcaacggccccagggcgtccagaacgggcttcaggcgctcccgaaggt

SEQ ID NO: 42 - DNA, 4457 bp, synthetic construct
  source 1..4457: mol_type = other DNA
ctcgggccgtctcttgggcttgatcggccttcttgcgcatctcacgcgctcctgcggcggcctgtagggcaggctcatacccctgccgaaccgcttttgtcagccggtcggccacggcttccggcgtctcaacgcgctttgagattcccagcttttcggccaatccctgcggtgcataggcgcgtggctcgaccgcttgcgggctgatggtgacgtggcccactggtggccgctccagggcctcgtagaacgcctgaatgcgcgtgtgacgtgccttgctgccctcgatgccccgttgcagccctagatcggccacagcggccgcaaacgtggtctggtcgcgggtcatctgcgctttgttgccgatgaactccttggccgacagcctgccgtcctgcgtcagcggcaccacgaacgcggtcatgtgcgggctggtttcgtcacggtggatgctggccgtcacgatgcgatccgccccgtacttgtccgccagccacttgtgcgccttctcgaagaacgccgcctgctgttcttggctggccgacttccaccattccgggctggccgtcatgacgtactcgaccgccaacacagcgtccttgcgccgcttctctggcagcaactcgcgcagtcggcccatcgcttcatcggtgctgctggccgcccagtgctcgttctctggcgtcctgctggcgtcagcgttgggcgtctcgcgctcgcggtaggcgtgcttgagactggccgccacgttgcccattttcgccagcttcttgcatcgcatgatcgcgtatgccgccatgcctgcccctcccttttggtgtccaaccggctcgacgggggcagcgcaaggcggtgcctccggcgggccactcaatgcttgagtatactcactagactttgcttcgcaaagtcgtgaccgcctacggcggctgcggcgccctacgggcttgctctccgggcttcgccctgcgcggtcgctgcgctcccttgccagcccgtggatatgtggacgatggccgcgagcggccaccggctggctcgcttcgctcggcccgtggacaaccctgctggacaagctgatggacaggctgcgcctgcccacgagcttgaccacagggattgcccaccggctacccagccttcgaccacatacccaccggctccaactgcgcggcctgcggccttgccccatcaatttttttaattttctctggggaaaagcctccggcctgcggcctgcgcgcttcgcttgccggttggacaccaagtggaaggcgggtcaaggctcgcgcagcgaccgcgcagcggcttggccttgacgcgcctggaacgacccaagcctatgcgagtgggggcagtcgaaggcgaagcccgcccgcctgccccccgagcctcacggcggcgagtgcgggggttccaagggggcagcgccaccttgggcaaggccgaaggccgcgcagtcgatcaacaagccccggaggggccactttttgccggagggggagccgcgccgaaggcgtgggggaaccccgcaggggtgcccttctttgggcaccaaagaactagatatagggcgaaatgcgaaagacttaaaaatcaacaacttaaaaaaggggggtacgcaacagctcattgcggcaccccccgcaatagctcattgcgtaggttaaagaaaatctgtaattgactgccacttttacgcaacgcataattgttgtcgcgctgccgaaaagttgcagctgattgcgcatggtgccgcaaccgtgcggcaccctaccgcatggagataagcatggccacgcagtccagagaaatcggcattcaagccaagaacaagcccggtcactgggtgcaaacggaacgcaaagcgcatgaggcgtgggccgggcttattgcgaggaaacccacggcggcaatgctgctgcatcacctcgtggcgcagatgggccaccagaacgccgtggtggtcagccagaagacactttccaagctcatcggacgttctttgcggacggtccaatacgcagtcaaggacttggtggccgagcgctggatctccgtcgtgaagctcaacggccccggcaccgtgtcggcctacgtggtcaatgaccgcgtggcgtggggccagccccgcgaccagttgcgcctgtcggtgttcagtgccgccgtggtggttgatcacgacgaccaggacgaatcgctgttggggcatggcgacctgcgccgcatcccgaccctgtatccgggcgagcagcaactaccgaccggccccggcgaggagccgcccagccagcccggcattccgggcatggaaccagacctgccagccttgaccgaaacggaggaatgggaacggcgcgggcagcagcgcctgccgatgcccgatgagccgtgttttctggacgatggcgagccgttggagccgccgacacgggtcacgctgccgcgccggtagggcatcaaataaaacgaaaggctcagtcgaaagactgggcctttcgttttatctgttgtttgtcggtgaacgctctcctgagtaggacaaatccgccgccctagattaattaagcccattgacaaggctctcgcggccaggtataattgcacgacctagggccaaagttcacttaaaaaggagatcaacaatgaaagcaattttcgtactgaaacatcttaatcatgctaaagaagttttctacttggactcctgttgatagatccagtaatgacctcagaactccatctggatttgttcagaacgctcggttgccgccgggcgttttttattggtgagaatccagattgcgttgcgctcactgcccgctttccagtcgggaaacctgtcgtgccagctgcattaatgaatcggccaacgcgcggggagaggcggtttgcgtattgggcgcatgcataaaaactgttgtaattcattaagcattctgccgacatggaagccatcacaaacggcatgatgaacctgaatcgccagcggcatcagcaccttgtcgccttgcgtataatatttgcccatgggggtgggcgaagaactccagcatgagatccccgcgctggaggatcatccagccggcgtcccggaaaacgattccgaagcccaacctttcatagaaggcggcggtggaatcgaaatctcgtgatggcaggttgggcgtcgcttggtcggtcatttcgaaccccagagtcccgctcagaagaactcgtcaagaaggcgatagaaggcgatgcgctgcgaatcgggagcggcgataccgtaaagcacgaggaagcggtcagcccattcgccgccaagctcttcagcaatatcacgggtagccaacgctatgtcctgatagcggtccgccacacccagccggccacagtcgatgaatccagaaaagcggccattttccaccatgatattcggcaagcaggcatcgccatgggtcacgacgagatcctcgccgtcgggcatgcgcgccttgagcctggcgaacagttcggctggcgcgagcccctgatgctcttcgtccagatcatcctgatcgacaagaccggcttccatccgagtacgtgctcgctcgatgcgatgtttcgcttggtggtcgaatgggcaggtagccggatcaagcgtatgcagccgccgcattgcatcagccatgatggatactttctcggcaggagcaaggtgagatgacaggagatcctgccccggcacttcgcccaatagcagccagtcccttcccgcttcagtgacaacgtcgagcacagctgcgcaaggaacgcccgtcgtggccagccacgatagccgcgctgcctcgtcctgcagttcattcagggcaccggacaggtcggtcttgacaaaaagaaccgggcgcccctgcgctgacagccggaacacggcggcatcagagcagccgattgtctgttgtgcccagtcatagccgaatagcctctccacccaagcggccggagaacctgcgtgcaatccatcttgttcaatcatgcgaaacgatcctcatcctgtctcttgatcagatcttgatcccctgcgccatcagatccttggcggcaagaaagccatccagtttactttgcagggcttcccaaccttaccagagggcgccccagctggcaattccggttcgcttgctgtccataaaaccgcccagtctagctatcgccatgtaagcccactgcaagctacctgctttctctttgcgcttgcgttttcccttgtccagatagcccagtagctgacattcatcccaggtggcacttttcggggaaatgtgcgcgcccgcgttcctgctggcgctgggcctgtttctggcgctggacttcccgctgttccgtcagcagcttttcgcccacggccttgatgatcgcggcggccttggcctgcatatcccgattcaacggccccagggcgtccagaacgggcttcaggcgctcccgaaggt

SEQ ID NO: 43 - DNA, 5642 bp, synthetic construct
  source 1..5642: mol_type = other DNA
ctcgggccgtctcttgggcttgatcggccttcttgcgcatctcacgcgctcctgcggcggcctgtagggcaggctcatacccctgccgaaccgcttttgtcagccggtcggccacggcttccggcgtctcaacgcgctttgagattcccagcttttcggccaatccctgcggtgcataggcgcgtggctcgaccgcttgcgggctgatggtgacgtggcccactggtggccgctccagggcctcgtagaacgcctgaatgcgcgtgtgacgtgccttgctgccctcgatgccccgttgcagccctagatcggccacagcggccgcaaacgtggtctggtcgcgggtcatctgcgctttgttgccgatgaactccttggccgacagcctgccgtcctgcgtcagcggcaccacgaacgcggtcatgtgcgggctggtttcgtcacggtggatgctggccgtcacgatgcgatccgccccgtacttgtccgccagccacttgtgcgccttctcgaagaacgccgcctgctgttcttggctggccgacttccaccattccgggctggccgtcatgacgtactcgaccgccaacacagcgtccttgcgccgcttctctggcagcaactcgcgcagtcggcccatcgcttcatcggtgctgctggccgcccagtgctcgttctctggcgtcctgctggcgtcagcgttgggcgtctcgcgctcgcggtaggcgtgcttgagactggccgccacgttgcccattttcgccagcttcttgcatcgcatgatcgcgtatgccgccatgcctgcccctcccttttggtgtccaaccggctcgacgggggcagcgcaaggcggtgcctccggcgggccactcaatgcttgagtatactcactagactttgcttcgcaaagtcgtgaccgcctacggcggctgcggcgccctacgggcttgctctccgggcttcgccctgcgcggtcgctgcgctcccttgccagcccgtggatatgtggacgatggccgcgagcggccaccggctggctcgcttcgctcggcccgtggacaaccctgctggacaagctgatggacaggctgcgcctgcccacgagcttgaccacagggattgcccaccggctacccagccttcgaccacatacccaccggctccaactgcgcggcctgcggccttgccccatcaatttttttaattttctctggggaaaagcctccggcctgcggcctgcgcgcttcgcttgccggttggacaccaagtggaaggcgggtcaaggctcgcgcagcgaccgcgcagcggcttggccttgacgcgcctggaacgacccaagcctatgcgagtgggggcagtcgaaggcgaagcccgcccgcctgccccccgagcctcacggcggcgagtgcgggggttccaagggggcagcgccaccttgggcaaggccgaaggccgcgcagtcgatcaacaagccccggaggggccactttttgccggagggggagccgcgccgaaggcgtgggggaaccccgcaggggtgcccttctttgggcaccaaagaactagatatagggcgaaatgcgaaagacttaaaaatcaacaacttaaaaaaggggggtacgcaacagctcattgcggcaccccccgcaatagctcattgcgtaggttaaagaaaatctgtaattgactgccacttttacgcaacgcataattgttgtcgcgctgccgaaaagttgcagctgattgcgcatggtgccgcaaccgtgcggcaccctaccgcatggagataagcatggccacgcagtccagagaaatcggcattcaagccaagaacaagcccggtcactgggtgcaaacggaacgcaaagcgcatgaggcgtgggccgggcttattgcgaggaaacccacggcggcaatgctgctgcatcacctcgtggcgcagatgggccaccagaacgccgtggtggtcagccagaagacactttccaagctcatcggacgttctttgcggacggtccaatacgcagtcaaggacttggtggccgagcgctggatctccgtcgtgaagctcaacggccccggcaccgtgtcggcctacgtggtcaatgaccgcgtggcgtggggccagccccgcgaccagttgcgcctgtcggtgttcagtgccgccgtggtggttgatcacgacgaccaggacgaatcgctgttggggcatggcgacctgcgccgcatcccgaccctgtatccgggcgagcagcaactaccgaccggccccggcgaggagccgcccagccagcccggcattccgggcatggaaccagacctgccagccttgaccgaaacggaggaatgggaacggcgcgggcagcagcgcctgccgatgcccgatgagccgtgttttctggacgatggcgagccgttggagccgccgacacgggtcacgctgccgcgccggtagggcatcaaataaaacgaaaggctcagtcgaaagactgggcctttcgttttatctgttgtttgtcggtgaacgctctcctgagtaggacaaatccgccgccctagattaattaagcccattgacaaggctctcgcggccaggtataattgcacgacctagggccaaagttcacttaaaaaggagatcaacaatgaaagcaattttcgtactgaaacatcttaatcatgctaaagaagttttctaatggccaaggtcttgttggaggaaatccgctcctcgcagcgcgccgaaggccccgccaccatcttggccatcggcacggctaccccggcgaacgtggtgtatcaggcagactacccagactactacttccgtattaccaagagcgagcatttgaccgaccttaaagaaaaatttaagcgtatgtgcgacaagtccatgattcgcaagcgctacatgcacctgagtgaagagatcttgaaggagaatccaaacatttgtgcctacatggcccccagtctcgacgctcgccaggacgtcgtagtcgtcgaggtgccgaagctgggcaaggaggcggcggtgaaggccatcaaggaatggggccaaccgaagtcgaagatcacccacctggtattttgcacgacgtccggcgtggacatgccgggtgcggactatcagctgactaagcttctgggcctgaggccaagcgtcaacaggctgatgatgtaccagcagggctgcttcgccggcggcacagtgctacgtctcgccaaagacttggccgaaaacaatcgtggtgcgcgcgtgctggtcgtgtgtagcgagatcaccgctgtgacgtttcgcggtccatccgagagccatctggacagcctggtcggccaggcgctgttcggtgatggcgccgccgcgatcatcgtgggcgcggacccggacccggccattgagcgccccctgttccagttggtgtcggccagccagaccatccttccagactcggagggcgcgattgacggccacctgcgggaagtgggactcaccttccacttactcaaagacgtaccaggcctgatctctaagaacatccataagtccctggtggaggccttcgtgccgctgggcatcagcgattggaacagtattttctggatcgcccaccctggtggtccggctatcctggaccaggtggaagccaagcttggcttggaaaaagagaagatgcgagccacccgccacgtgctgagcgaatacggcaacatgtccagcgcctgcgtgctgttcatcctcgacgagatgcgacgtcgcagcgcagaagaggggaaagccaccacaggtgagggcctcgagtggggtgtgttgttcggtttcgggccgggccttaccgtggagaccgtggtgctgcacagtcttccgataagtacccgttgacttggactcctgttgatagatccagtaatgacctcagaactccatctggatttgttcagaacgctcggttgccgccgggcgttttttattggtgagaatccagattgcgttgcgctcactgcccgctttccagtcgggaaacctgtcgtgccagctgcattaatgaatcggccaacgcgcggggagaggcggtttgcgtattgggcgcatgcataaaaactgttgtaattcattaagcattctgccgacatggaagccatcacaaacggcatgatgaacctgaatcgccagcggcatcagcaccttgtcgccttgcgtataatatttgcccatgggggtgggcgaagaactccagcatgagatccccgcgctggaggatcatccagccggcgtcccggaaaacgattccgaagcccaacctttcatagaaggcggcggtggaatcgaaatctcgtgatggcaggttgggcgtcgcttggtcggtcatttcgaaccccagagtcccgctcagaagaactcgtcaagaaggcgatagaaggcgatgcgctgcgaatcgggagcggcgataccgtaaagcacgaggaagcggtcagcccattcgccgccaagctcttcagcaatatcacgggtagccaacgctatgtcctgatagcggtccgccacacccagccggccacagtcgatgaatccagaaaagcggccattttccaccatgatattcggcaagcaggcatcgccatgggtcacgacgagatcctcgccgtcgggcatgcgcgccttgagcctggcgaacagttcggctggcgcgagcccctgatgctcttcgtccagatcatcctgatcgacaagaccggcttccatccgagtacgtgctcgctcgatgcgatgtttcgcttggtggtcgaatgggcaggtagccggatcaagcgtatgcagccgccgcattgcatcagccatgatggatactttctcggcaggagcaaggtgagatgacaggagatcctgccccggcacttcgcccaatagcagccagtcccttcccgcttcagtgacaacgtcgagcacagctgcgcaaggaacgcccgtcgtggccagccacgatagccgcgctgcctcgtcctgcagttcattcagggcaccggacaggtcggtcttgacaaaaagaaccgggcgcccctgcgctgacagccggaacacggcggcatcagagcagccgattgtctgttgtgcccagtcatagccgaatagcctctccacccaagcggccggagaacctgcgtgcaatccatcttgttcaatcatgcgaaacgatcctcatcctgtctcttgatcagatcttgatcccctgcgccatcagatccttggcggcaagaaagccatccagtttactttgcagggcttcccaaccttaccagagggcgccccagctggcaattccggttcgcttgctgtccataaaaccgcccagtctagctatcgccatgtaagcccactgcaagctacctgctttctctttgcgcttgcgttttcccttgtccagatagcccagtagctgacattcatcccaggtggcacttttcggggaaatgtgcgcgcccgcgttcctgctggcgctgggcctgtttctggcgctggacttcccgctgttccgtcagcagcttttcgcccacggccttgatgatcgcggcggccttggcctgcatatcccgattcaacggccccagggcgtccagaacgggcttcaggcgctcccgaaggt

SEQ ID NO: 44 - DNA, 5642 bp, synthetic construct
  source 1..5642: mol_type = other DNA
ctcgggccgtctcttgggcttgatcggccttcttgcgcatctcacgcgctcctgcggcggcctgtagggcaggctcatacccctgccgaaccgcttttgtcagccggtcggccacggcttccggcgtctcaacgcgctttgagattcccagcttttcggccaatccctgcggtgcataggcgcgtggctcgaccgcttgcgggctgatggtgacgtggcccactggtggccgctccagggcctcgtagaacgcctgaatgcgcgtgtgacgtgccttgctgccctcgatgccccgttgcagccctagatcggccacagcggccgcaaacgtggtctggtcgcgggtcatctgcgctttgttgccgatgaactccttggccgacagcctgccgtcctgcgtcagcggcaccacgaacgcggtcatgtgcgggctggtttcgtcacggtggatgctggccgtcacgatgcgatccgccccgtacttgtccgccagccacttgtgcgccttctcgaagaacgccgcctgctgttcttggctggccgacttccaccattccgggctggccgtcatgacgtactcgaccgccaacacagcgtccttgcgccgcttctctggcagcaactcgcgcagtcggcccatcgcttcatcggtgctgctggccgcccagtgctcgttctctggcgtcctgctggcgtcagcgttgggcgtctcgcgctcgcggtaggcgtgcttgagactggccgccacgttgcccattttcgccagcttcttgcatcgcatgatcgcgtatgccgccatgcctgcccctcccttttggtgtccaaccggctcgacgggggcagcgcaaggcggtgcctccggcgggccactcaatgcttgagtatactcactagactttgcttcgcaaagtcgtgaccgcctacggcggctgcggcgccctacgggcttgctctccgggcttcgccctgcgcggtcgctgcgctcccttgccagcccgtggatatgtggacgatggccgcgagcggccaccggctggctcgcttcgctcggcccgtggacaaccctgctggacaagctgatggacaggctgcgcctgcccacgagcttgaccacagggattgcccaccggctacccagccttcgaccacatacccaccggctccaactgcgcggcctgcggccttgccccatcaatttttttaattttctctggggaaaagcctccggcctgcggcctgcgcgcttcgcttgccggttggacaccaagtggaaggcgggtcaaggctcgcgcagcgaccgcgcagcggcttggccttgacgcgcctggaacgacccaagcctatgcgagtgggggcagtcgaaggcgaagcccgcccgcctgccccccgagcctcacggcggcgagtgcgggggttccaagggggcagcgccaccttgggcaaggccgaaggccgcgcagtcgatcaacaagccccggaggggccactttttgccggagggggagccgcgccgaaggcgtgggggaaccccgcaggggtgcccttctttgggcaccaaagaactagatatagggcgaaatgcgaaagacttaaaaatcaacaacttaaaaaaggggggtacgcaacagctcattgcggcaccccccgcaatagctcattgcgtaggttaaagaaaatctgtaattgactgccacttttacgcaacgcataattgttgtcgcgctgccgaaaagttgcagctgattgcgcatggtgccgcaaccgtgcggcaccctaccgcatggagataagcatggccacgcagtccagagaaatcggcattcaagccaagaacaagcccggtcactgggtgcaaacggaacgcaaagcgcatgaggcgtgggccgggcttattgcgaggaaacccacggcggcaatgctgctgcatcacctcgtggcgcagatgggccaccagaacgccgtggtggtcagccagaagacactttccaagctcatcggacgttctttgcggacggtccaatacgcagtcaaggacttggtggccgagcgctggatctccgtcgtgaagctcaacggccccggcaccgtgtcggcctacgtggtcaatgaccgcgtggcgtggggccagccccgcgaccagttgcgcctgtcggtgttcagtgccgccgtggtggttgatcacgacgaccaggacgaatcgctgttggggcatggcgacctgcgccgcatcccgaccctgtatccgggcgagcagcaactaccgaccggccccggcgaggagccgcccagccagcccggcattccgggcatggaaccagacctgccagccttgaccgaaacggaggaatgggaacggcgcgggcagcagcgcctgccgatgcccgatgagccgtgttttctggacgatggcgagccgttggagccgccgacacgggtcacgctgccgcgccggtagggcatcaaataaaacgaaaggctcagtcgaaagactgggcctttcgttttatctgttgtttgtcggtgaacgctctcctgagtaggacaaatccgccgccctagattaattaagcccattgacaaggctctcgcggccaggtataattgcacgacctagggccaaagttcacttaaaaaggagatcaacaatgaaagcaattttcgtactgaaacatcttaatcatgctaaagaagttttctaatggccaaggtcttgttggaggaaatccgctcctcgcagcgcgccgaaggccccgccaccatcttggccatcggcacggctaccccggcgaacgtggtgtatcaggcagactacccagactactacttccgtattaccaagagcgagcatttgaccgaccttaaagaaaaatttaagcgtatgtgcgacaagtccatgattcgcaagcgctacatgcacctgagtgaagagatcttgaaggagaatccaaacatttgtgcctacatggcccccagtctcgacgctcgccaggacgtcgtagtcgtcgaggtgccgaagctgggcaaggaggcggcggtgaaggccatcaaggaatggggccaaccgaagtcgaagatcacccacctggtattttgcacgacgtccggcgtggacatgccgggtgcggactatcagctgactaagcttctgggcctgaggccaagcgtcaacaggctgatgatgtaccagcagggctgcttcgccggcggcacagtgctacgtctcgccaaagacttggccgaaaacaatcgtggtgcgcgcgtgctggtcgtgtgtagcgagatcaccgctgtgacgtttcgcggtccatccgagagccatctggacagcctggtcggccaggcgctgttcggtgatggcgccgccgcgatcatcgtgggcgcggacccggacccggccattgagcgccccctgttccagttggtgtcggccagccagaccatccttccagactcggagggcgcgattgacggccacctgcgggaagtgggactcaccttccacttactcaaagacgtaccaggcctgatctctaagaacatccataagtccctggtggaggccttcgccccgctgggcatcagcgattggaacagtattttctggatcgcccaccctggtggtccggctatcctggaccaggtggaagccaagcttggcttggaaaaagagaagatgcgagccacccgccacgtgctgagcgaatacggcaacatgtccagcgcctgcgtgctgttcatcctcgacgagatgcgacgtcgcagcgcagaagaggggaaagccaccacaggtgagggcctcgagtggggtgtgttgttcggtttcgggccgggccttaccgtggagaccgtggtgctgcacagtcttccgataagtacccgttgacttggactcctgttgatagatccagtaatgacctcagaactccatctggatttgttcagaacgctcggttgccgccgggcgttttttattggtgagaatccagattgcgttgcgctcactgcccgctttccagtcgggaaacctgtcgtgccagctgcattaatgaatcggccaacgcgcggggagaggcggtttgcgtattgggcgcatgcataaaaactgttgtaattcattaagcattctgccgacatggaagccatcacaaacggcatgatgaacctgaatcgccagcggcatcagcaccttgtcgccttgcgtataatatttgcccatgggggtgggcgaagaactccagcatgagatccccgcgctggaggatcatccagccggcgtcccggaaaacgattccgaagcccaacctttcatagaaggcggcggtggaatcgaaatctcgtgatggcaggttgggcgtcgcttggtcggtcatttcgaaccccagagtcccgctcagaagaactcgtcaagaaggcgatagaaggcgatgcgctgcgaatcgggagcggcgataccgtaaagcacgaggaagcggtcagcccattcgccgccaagctcttcagcaatatcacgggtagccaacgctatgtcctgatagcggtccgccacacccagccggccacagtcgatgaatccagaaaagcggccattttccaccatgatattcggcaagcaggcatcgccatgggtcacgacgagatcctcgccgtcgggcatgcgcgccttgagcctggcgaacagttcggctggcgcgagcccctgatgctcttcgtccagatcatcctgatcgacaagaccggcttccatccgagtacgtgctcgctcgatgcgatgtttcgcttggtggtcgaatgggcaggtagccggatcaagcgtatgcagccgccgcattgcatcagccatgatggatactttctcggcaggagcaaggtgagatgacaggagatcctgccccggcacttcgcccaatagcagccagtcccttcccgcttcagtgacaacgtcgagcacagctgcgcaaggaacgcccgtcgtggccagccacgatagccgcgctgcctcgtcctgcagttcattcagggcaccggacaggtcggtcttgacaaaaagaaccgggcgcccctgcgctgacagccggaacacggcggcatcagagcagccgattgtctgttgtgcccagtcatagccgaatagcctctccacccaagcggccggagaacctgcgtgcaatccatcttgttcaatcatgcgaaacgatcctcatcctgtctcttgatcagatcttgatcccctgcgccatcagatccttggcggcaagaaagccatccagtttactttgcagggcttcccaaccttaccagagggcgccccagctggcaattccggttcgcttgctgtccataaaaccgcccagtctagctatcgccatgtaagcccactgcaagctacctgctttctctttgcgcttgcgttttcccttgtccagatagcccagtagctgacattcatcccaggtggcacttttcggggaaatgtgcgcgcccgcgttcctgctggcgctgggcctgtttctggcgctggacttcccgctgttccgtcagcagcttttcgcccacggccttgatgatcgcggcggccttggcctgcatatcccgattcaacggccccagggcgtccagaacgggcttcaggcgctcccgaaggt

SEQ ID NO: 45 - DNA, 5642 bp, synthetic construct
  source 1..5642: mol_type = other DNA
ctcgggccgtctcttgggcttgatcggccttcttgcgcatctcacgcgctcctgcggcggcctgtagggcaggctcatacccctgccgaaccgcttttgtcagccggtcggccacggcttccggcgtctcaacgcgctttgagattcccagcttttcggccaatccctgcggtgcataggcgcgtggctcgaccgcttgcgggctgatggtgacgtggcccactggtggccgctccagggcctcgtagaacgcctgaatgcgcgtgtgacgtgccttgctgccctcgatgccccgttgcagccctagatcggccacagcggccgcaaacgtggtctggtcgcgggtcatctgcgctttgttgccgatgaactccttggccgacagcctgccgtcctgcgtcagcggcaccacgaacgcggtcatgtgcgggctggtttcgtcacggtggatgctggccgtcacgatgcgatccgccccgtacttgtccgccagccacttgtgcgccttctcgaagaacgccgcctgctgttcttggctggccgacttccaccattccgggctggccgtcatgacgtactcgaccgccaacacagcgtccttgcgccgcttctctggcagcaactcgcgcagtcggcccatcgcttcatcggtgctgctggccgcccagtgctcgttctctggcgtcctgctggcgtcagcgttgggcgtctcgcgctcgcggtaggcgtgcttgagactggccgccacgttgcccattttcgccagcttcttgcatcgcatgatcgcgtatgccgccatgcctgcccctcccttttggtgtccaaccggctcgacgggggcagcgcaaggcggtgcctccggcgggccactcaatgcttgagtatactcactagactttgcttcgcaaagtcgtgaccgcctacggcggctgcggcgccctacgggcttgctctccgggcttcgccctgcgcggtcgctgcgctcccttgccagcccgtggatatgtggacgatggccgcgagcggccaccggctggctcgcttcgctcggcccgtggacaaccctgctggacaagctgatggacaggctgcgcctgcccacgagcttgaccacagggattgcccaccggctacccagccttcgaccacatacccaccggctccaactgcgcggcctgcggccttgccccatcaatttttttaattttctctggggaaaagcctccggcctgcggcctgcgcgcttcgcttgccggttggacaccaagtggaaggcgggtcaaggctcgcgcagcgaccgcgcagcggcttggccttgacgcgcctggaacgacccaagcctatgcgagtgggggcagtcgaaggcgaagcccgcccgcctgccccccgagcctcacggcggcgagtgcgggggttccaagggggcagcgccaccttgggcaaggccgaaggccgcgcagtcgatcaacaagccccggaggggccactttttgccggagggggagccgcgccgaaggcgtgggggaaccccgcaggggtgcccttctttgggcaccaaagaactagatatagggcgaaatgcgaaagacttaaaaatcaacaacttaaaaaaggggggtacgcaacagctcattgcggcaccccccgcaatagctcattgcgtaggttaaagaaaatctgtaattgactgccacttttacgcaacgcataattgttgtcgcgctgccgaaaagttgcagctgattgcgcatggtgccgcaaccgtgcggcaccctaccgcatggagataagcatggccacgcagtccagagaaatcggcattcaagccaagaacaagcccggtcactgggtgcaaacggaacgcaaagcgcatgaggcgtgggccgggcttattgcgaggaaacccacggcggcaatgctgctgcatcacctcgtggcgcagatgggccaccagaacgccgtggtggtcagccagaagacactttccaagctcatcggacgttctttgcggacggtccaatacgcagtcaaggacttggtggccgagcgctggatctccgtcgtgaagctcaacggccccggcaccgtgtcggcctacgtggtcaatgaccgcgtggcgtggggccagccccgcgaccagttgcgcctgtcggtgttcagtgccgccgtggtggttgatcacgacgaccaggacgaatcgctgttggggcatggcgacctgcgccgcatcccgaccctgtatccgggcgagcagcaactaccgaccggccccggcgaggagccgcccagccagcccggcattccgggcatggaaccagacctgccagccttgaccgaaacggaggaatgggaacggcgcgggcagcagcgcctgccgatgcccgatgagccgtgttttctggacgatggcgagccgttggagccgccgacacgggtcacgctgccgcgccggtagggcatcaaataaaacgaaaggctcagtcgaaagactgggcctttcgttttatctgttgtttgtcggtgaacgctctcctgagtaggacaaatccgccgccctagattaattaagcccattgacaaggctctcgcggccaggtataattgcacgacctagggccaaagttcacttaaaaaggagatcaacaatgaaagcaattttcgtactgaaacatcttaatcatgctaaagaagttttctaatggccaaggtcttgttggaggaaatccgctcctcgcagcgcgccgaaggccccgccaccatcttggccatcggcacggctaccccggcgaacgtggtgtatcaggcagactacgcagactactacttccgtattaccaagagcgagcatttgaccgaccttaaagaaaaatttaagcgtatgtgcgacaagtccatgattcgcaagcgctacatgcacctgagtgaagagatcttgaaggagaatccaaacatttgtgcctacatggcccccagtctcgacgctcgccaggacgtcgtagtcgtcgaggtgccgaagctgggcaaggaggcggcggtgaaggccatcaaggaatggggccaaccgaagtcgaagatcacccacctggtattttgcacgacgtccggcgtggacatgccgggtgcggactatcagctgactaagcttctgggcctgaggccaagcgtcaacaggctgatgatgtaccagcagggctgcttcgccggcggcacagtgctacgtctcgccaaagacttggccgaaaacaatcgtggtgcgcgcgtgctggtcgtgtgtagcgagatcaccgctgtgacgtttcgcggtccatccgagagccatctggacagcctggtcggccaggcgctgttcggtgatggcgccgccgcgatcatcgtgggcgcggacccggacccggccattgagcgccccctgttccagttggtgtcggccagccagaccatccttccagactcggagggcgcgattgacggccacctgcgggaagtgggactcaccttccacttactcaaagacgtaccaggcctgatctctaagaacatccataagtccctggtggaggccttcgtgccgctgggcatcagcgattggaacagtattttctggatcgcccaccctggtggtccggctatcctggaccaggtggaagccaagcttggcttggaaaaagagaagatgcgagccacccgccacgtgctgagcgaatacggcaacatgtccagcgcctgcgtgctgttcatcctcgacgagatgcgacgtcgcagcgcagaagaggggaaagccaccacaggtgagggcctcgagtggggtgtgttgttcggtttcgggccgggccttaccgtggagaccgtggtgctgcacagtcttccgataagtacccgttgacttggactcctgttgatagatccagtaatgacctcagaactccatctggatttgttcagaacgctcggttgccgccgggcgttttttattggtgagaatccagattgcgttgcgctcactgcccgctttccagtcgggaaacctgtcgtgccagctgcattaatgaatcggccaacgcgcggggagaggcggtttgcgtattgggcgcatgcataaaaactgttgtaattcattaagcattctgccgacatggaagccatcacaaacggcatgatgaacctgaatcgccagcggcatcagcaccttgtcgccttgcgtataatatttgcccatgggggtgggcgaagaactccagcatgagatccccgcgctggaggatcatccagccggcgtcccggaaaacgattccgaagcccaacctttcatagaaggcggcggtggaatcgaaatctcgtgatggcaggttgggcgtcgcttggtcggtcatttcgaaccccagagtcccgctcagaagaactcgtcaagaaggcgatagaaggcgatgcgctgcgaatcgggagcggcgataccgtaaagcacgaggaagcggtcagcccattcgccgccaagctcttcagcaatatcacgggtagccaacgctatgtcctgatagcggtccgccacacccagccggccacagtcgatgaatccagaaaagcggccattttccaccatgatattcggcaagcaggcatcgccatgggtcacgacgagatcctcgccgtcgggcatgcgcgccttgagcctggcgaacagttcggctggcgcgagcccctgatgctcttcgtccagatcatcctgatcgacaagaccggcttccatccgagtacgtgctcgctcgatgcgatgtttcgcttggtggtcgaatgggcaggtagccggatcaagcgtatgcagccgccgcattgcatcagccatgatggatactttctcggcaggagcaaggtgagatgacaggagatcctgccccggcacttcgcccaatagcagccagtcccttcccgcttcagtgacaacgtcgagcacagctgcgcaaggaacgcccgtcgtggccagccacgatagccgcgctgcctcgtcctgcagttcattcagggcaccggacaggtcggtcttgacaaaaagaaccgggcgcccctgcgctgacagccggaacacggcggcatcagagcagccgattgtctgttgtgcccagtcatagccgaatagcctctccacccaagcggccggagaacctgcgtgcaatccatcttgttcaatcatgcgaaacgatcctcatcctgtctcttgatcagatcttgatcccctgcgccatcagatccttggcggcaagaaagccatccagtttactttgcagggcttcccaaccttaccagagggcgccccagctggcaattccggttcgcttgctgtccataaaaccgcccagtctagctatcgccatgtaagcccactgcaagctacctgctttctctttgcgcttgcgttttcccttgtccagatagcccagtagctgacattcatcccaggtggcacttttcggggaaatgtgcgcgcccgcgttcctgctggcgctgggcctgtttctggcgctggacttcccgctgttccgtcagcagcttttcgcccacggccttgatgatcgcggcggccttggcctgcatatcccgattcaacggccccagggcgtccagaacgggcttcaggcgctcccgaaggt

SEQ ID NO: 46 - DNA, 5642 bp, synthetic construct
  source 1..5642: mol_type = other DNA
ctcgggccgtctcttgggcttgatcggccttcttgcgcatctcacgcgctcctgcggcggcctgtagggcaggctcatacccctgccgaaccgcttttgtcagccggtcggccacggcttccggcgtctcaacgcgctttgagattcccagcttttcggccaatccctgcggtgcataggcgcgtggctcgaccgcttgcgggctgatggtgacgtggcccactggtggccgctccagggcctcgtagaacgcctgaatgcgcgtgtgacgtgccttgctgccctcgatgccccgttgcagccctagatcggccacagcggccgcaaacgtggtctggtcgcgggtcatctgcgctttgttgccgatgaactccttggccgacagcctgccgtcctgcgtcagcggcaccacgaacgcggtcatgtgcgggctggtttcgtcacggtggatgctggccgtcacgatgcgatccgccccgtacttgtccgccagccacttgtgcgccttctcgaagaacgccgcctgctgttcttggctggccgacttccaccattccgggctggccgtcatgacgtactcgaccgccaacacagcgtccttgcgccgcttctctggcagcaactcgcgcagtcggcccatcgcttcatcggtgctgctggccgcccagtgctcgttctctggcgtcctgctggcgtcagcgttgggcgtctcgcgctcgcggtaggcgtgcttgagactggccgccacgttgcccattttcgccagcttcttgcatcgcatgatcgcgtatgccgccatgcctgcccctcccttttggtgtccaaccggctcgacgggggcagcgcaaggcggtgcctccggcgggccactcaatgcttgagtatactcactagactttgcttcgcaaagtcgtgaccgcctacggcggctgcggcgccctacgggcttgctctccgggcttcgccctgcgcggtcgctgcgctcccttgccagcccgtggatatgtggacgatggccgcgagcggccaccggctggctcgcttcgctcggcccgtggacaaccctgctggacaagctgatggacaggctgcgcctgcccacgagcttgaccacagggattgcccaccggctacccagccttcgaccacatacccaccggctccaactgcgcggcctgcggccttgccccatcaatttttttaattttctctggggaaaagcctccggcctgcggcctgcgcgcttcgcttgccggttggacaccaagtggaaggcgggtcaaggctcgcgcagcgaccgcgcagcggcttggccttgacgcgcctggaacgacccaagcctatgcgagtgggggcagtcgaaggcgaagcccgcccgcctgccccccgagcctcacggcggcgagtgcgggggttccaagggggcagcgccaccttgggcaaggccgaaggccgcgcagtcgatcaacaagccccggaggggccactttttgccggagggggagccgcgccgaaggcgtgggggaaccccgcaggggtgcccttctttgggcaccaaagaactagatatagggcgaaatgcgaaagacttaaaaatcaacaacttaaaaaaggggggtacgcaacagctcattgcggcaccccccgcaatagctcattgcgtaggttaaagaaaatctgtaattgactgccacttttacgcaacgcataattgttgtcgcgctgccgaaaagttgcagctgattgcgcatggtgccgcaaccgtgcggcaccctaccgcatggagataagcatggccacgcagtccagagaaatcggcattcaagccaagaacaagcccggtcactgggtgcaaacggaacgcaaagcgcatgaggcgtgggccgggcttattgcgaggaaacccacggcggcaatgctgctgcatcacctcgtggcgcagatgggccaccagaacgccgtggtggtcagccagaagacactttccaagctcatcggacgttctttgcggacggtccaatacgcagtcaaggacttggtggccgagcgctggatctccgtcgtgaagctcaacggccccggcaccgtgtcggcctacgtggtcaatgaccgcgtggcgtggggccagccccgcgaccagttgcgcctgtcggtgttcagtgccgccgtggtggttgatcacgacgaccaggacgaatcgctgttggggcatggcgacctgcgccgcatcccgaccctgtatccgggcgagcagcaactaccgaccggccccggcgaggagccgcccagccagcccggcattccgggcatggaaccagacctgccagccttgaccgaaacggaggaatgggaacggcgcgggcagcagcgcctgccgatgcccgatgagccgtgttttctggacgatggcgagccgttggagccgccgacacgggtcacgctgccgcgccggtagggcatcaaataaaacgaaaggctcagtcgaaagactgggcctttcgttttatctgttgtttgtcggtgaacgctctcctgagtaggacaaatccgccgccctagattaattaagcccattgacaaggctctcgcggccaggtataattgcacgacctagggccaaagttcacttaaaaaggagatcaacaatgaaagcaattttcgtactgaaacatcttaatcatgctaaagaagttttctaatggccaaggtcttgttggaggaaatccgctcctcgcagcgcgccgatggccccgccaccatcttggccatcggcacggctaccccggcgaacgtggtgtatcaggcagactacccagactactacttccgtattaccaagagcgagcatttgaccgaccttaaagaaaaatttaagcgtatgtgcgacaagtccatgattcgcaagcgctacatgcacctgagtgaagagatcttgaaggagaatccaaacatttgtgcctacatggcccccagtctcgacgctcgccaggacgtcgtagtcgtcgaggtgccgaagctgggcaaggaggcggcggtgaaggccatcaaggaatggggccaaccgaagtcgaagatcacccacctggtattttgcacgacgtccggcgtggacatgccgggtgcggactatcagctgactaagcttctgggcctgaggccaagcgtcaacaggctgatgatgtaccagcagggctgcttcgccggcggcacagtgctacgtctcgccaaagacttggccgaaaacaatcgtggtgcgcgcgtgctggtcgtgtgtagcgagatcaccgctgtgacgtttcgcggtccatccgagagccatctggacagcctggtcggccaggcgctgttcggtgatggcgccgccgcgatcatcgtgggcgcggacccggacccggccattgagcgccccctgttccagttggtgtcggccagccagaccatccttccagactcggagggcgcgattgacggccacctgcgggaagtgggactcaccttccacttactcaaagacgtaccaggcctgatctctaagaacatccataagtccctggtggaggccttcgtgccgctgggcatcagcgattggaacagtattttctggatcgcccaccctggtggtccggctatcctggaccaggtggaagccaagcttggcttggaaaaagagaagatgcgagccacccgccacgtgctgagcgaatacggcaacatgtccagcgcctgcgtgctgttcatcctcgacgagatgcgacgtcgcagcgcagaagaggggaaagccaccacaggtgagggcctcgagtggggtgtgttgttcggtttcgggccgggccttaccgtggagaccgtggtgctgcacagtcttccgataagtacccgttgacttggactcctgttgatagatccagtaatgacctcagaactccatctggatttgttcagaacgctcggttgccgccgggcgttttttattggtgagaatccagattgcgttgcgctcactgcccgctttccagtcgggaaacctgtcgtgccagctgcattaatgaatcggccaacgcgcggggagaggcggtttgcgtattgggcgcatgcataaaaactgttgtaattcattaagcattctgccgacatggaagccatcacaaacggcatgatgaacctgaatcgccagcggcatcagcaccttgtcgccttgcgtataatatttgcccatgggggtgggcgaagaactccagcatgagatccccgcgctggaggatcatccagccggcgtcccggaaaacgattccgaagcccaacctttcatagaaggcggcggtggaatcgaaatctcgtgatggcaggttgggcgtcgcttggtcggtcatttcgaaccccagagtcccgctcagaagaactcgtcaagaaggcgatagaaggcgatgcgctgcgaatcgggagcggcgataccgtaaagcacgaggaagcggtcagcccattcgccgccaagctcttcagcaatatcacgggtagccaacgctatgtcctgatagcggtccgccacacccagccggccacagtcgatgaatccagaaaagcggccattttccaccatgatattcggcaagcaggcatcgccatgggtcacgacgagatcctcgccgtcgggcatgcgcgccttgagcctggcgaacagttcggctggcgcgagcccctgatgctcttcgtccagatcatcctgatcgacaagaccggcttccatccgagtacgtgctcgctcgatgcgatgtttcgcttggtggtcgaatgggcaggtagccggatcaagcgtatgcagccgccgcattgcatcagccatgatggatactttctcggcaggagcaaggtgagatgacaggagatcctgccccggcacttcgcccaatagcagccagtcccttcccgcttcagtgacaacgtcgagcacagctgcgcaaggaacgcccgtcgtggccagccacgatagccgcgctgcctcgtcctgcagttcattcagggcaccggacaggtcggtcttgacaaaaagaaccgggcgcccctgcgctgacagccggaacacggcggcatcagagcagccgattgtctgttgtgcccagtcatagccgaatagcctctccacccaagcggccggagaacctgcgtgcaatccatcttgttcaatcatgcgaaacgatcctcatcctgtctcttgatcagatcttgatcccctgcgccatcagatccttggcggcaagaaagccatccagtttactttgcagggcttcccaaccttaccagagggcgccccagctggcaattccggttcgcttgctgtccataaaaccgcccagtctagctatcgccatgtaagcccactgcaagctacctgctttctctttgcgcttgcgttttcccttgtccagatagcccagtagctgacattcatcccaggtggcacttttcggggaaatgtgcgcgcccgcgttcctgctggcgctgggcctgtttctggcgctggacttcccgctgttccgtcagcagcttttcgcccacggccttgatgatcgcggcggccttggcctgcatatcccgattcaacggccccagggcgtccagaacgggcttcaggcgctcccgaaggt